European Patent Application EP 4 450 127 A2, published October 23, 2024. Title: METHOD OF USING A GIP/GLP1 CO-AGONIST FOR DIABETES. Applicant: Eli Lilly and Company. Application EP. The sequence listing filed with the application follows.

SEQUENCE LISTING (145 sequences)

SEQ ID NO: 1 - protein, 42 aa, Homo sapiens
YAEGTFISDYSIAMDKIHQQDFVNWLLAQKGKKNDWKHNITQ

SEQ ID NO: 2 - protein, 30 aa, Homo sapiens
  MOD_RES 30: note = AMIDATION
HAEGTFTSDVSSYLEGQAAKEFIAWLVKGR

SEQ ID NO: 3 - protein, 31 aa, synthetic construct
  REGION 1..31: note = Synthetic construct; Formula I
  VARIANT 1: note = Xaa at position 1 is selected from the group consisting of Y, H, D-Tyr, F, desH, and desY, or Xaa at position 1 and Xaa at position 2 combine to form desH-psi[NHCO]-Aib
  MOD_RES 1: note = The N-terminus of Xaa at position 1 is modified with R1, wherein the modification is selected from the group consisting of Ac and absent.
  VARIANT 2: note = Xaa at position 2 is selected from the group consisting of Aib, alpha-MeP, A, P, and D-Ala, or Xaa at position 1 combines with Xaa at position 2 to form desH-psi[NHCO]-Aib
  VARIANT 3: note = Xaa at position 3 is selected from the group of E, N, Aad, and cTA
  VARIANT 6: note = Xaa at position 6 is selected from the group consisting of F, alpha-MeF, and alpha-MeF(2F)
  VARIANT 10: note = Xaa at position 10 is selected from the group consisting of A, L, H, 3Pal, 4Pal, V, Y, E, alpha-MeF, alpha-MeF(2F), I, alpha-MeY, Q, D-His, D-Tyr, cTA, and K
  VARIANT 10: note = when Xaa at position 10 is K, then K is chemically modified by conjugation of the epsilon-amino group of the K side chain with (2-[2-(2-amino-ethoxy)-ethoxy]-acetyl)2-(gamma-Glu)-CO-(CH2)q-CO2 H
  REGION 10..31: note = MISC_FEATURE - When Xaa is K(2-[2-(2-amino-ethoxy)-ethoxy]-acetyl)2-(gamma-Glu)-CO-(CH2)q-CO 2H at positions 10, 12, 13, 14, 16, 17, 19, 20, 21, 23, 24, 26, 27, 28, 29, 30 or 31, q is 14, 15, 16, 17, 18, 19 or 20.
  VARIANT 11: note = Xaa at position 11 is selected from the group consisting of S, alpha-MeS, or D-Ser
  VARIANT 12: note = Xaa at position 12 is selected from the group consisting of I, S, D-Ile, and K
  MOD_RES 12: note = when Xaa at position 12 is K, then K is chemically modified by conjugation of the epsilon-amino group of the K side chain with (2-[2-(2-amino-ethoxy)-ethoxy]-acetyl)2-(gamma-Glu)-CO-(CH2)q-CO2 H
  VARIANT 13: note = Xaa at position 13 is selected from the group consisting of Nle, Aib, L, alpha-MeL, and K
  MOD_RES 13: note = when Xaa at position 13 is K, then K is chemically modified by conjugation of the epsilon-amino group of the K side chain with (2-[2-(2-amino-ethoxy)-ethoxy]-acetyl)2-(gamma-Glu)-CO-(CH2)q-CO2 H
  VARIANT 14: note = Xaa at position 14 is selected from the group consisting of L and K, wherein K is conjugated to a C16-C22 fatty acid wherein said fatty acid is optionally conjugated to said K via a linker
  VARIANT 16: note = Xaa at position 16 is selected from the group consisting of E, Orn, Dab, Dap, S, T, H, Aib, alpha-MeK, R, and K
  MOD_RES 16: note = when Xaa at position 16 is K, then K is optionally chemically modified by conjugation of the epsilon-amino group of the K side chain with (2-[2-(2-amino-ethoxy)-ethoxy]-acetyl)2 -(gamma-Glu)-CO-(CH2)q-CO2H
  VARIANT 17: note = Xaa at position 17 is selected from the group consisting of K, Q, I, and an amino acid conjugated to a C16-C22 fatty acid wherein said fatty acid is optionally conjugated to said amino acid via a linker
  VARIANT 19: note = Xaa at position 19 is selected from the group consisting of Q, A, and K
  MOD_RES 19: note = when Xaa at position 19 is K, then K is chemically modified by conjugation of the epsilon-amino group of the K side chain with (2-[2-(2-amino-ethoxy)-ethoxy]-acetyl)2 -(gamma-Glu)-CO-(CH2)q-CO2H
  VARIANT 20: note = Xaa at position 20 is selected from the group consisting of Aib, Q, H, R, K, and alpha-MeK
  MOD_RES 20: note = when Xaa at position 20 is K, then K is optionally chemically modified by conjugation of the epsilon-amino group of the K side chain with (2-[2-(2-amino-ethoxy)-ethoxy]-acetyl)2 -(gamma-Glu)-CO-(CH2)q-CO2H
  VARIANT 21: note = Xaa at position 21 is selected from the group consisting of H, Aad, D, Aib, T, A, E, I, and K
  MOD_RES 21: note = when Xaa at position 21 is K, then K is chemically modified by conjugation of the epsilon-amino group of the K side chain with K(2-[2-(2-amino-ethoxy)-ethoxy]-acetyl)2-(gamma-Glu)-CO-(CH2)q-CO 2H
  VARIANT 22: note = Xaa at position 22 is selected from the group consisting of F and alpha-MeF
  VARIANT 23: note = Xaa at position 23 is selected from the group consisting of I, L, A, G, F, H, E, V, and K
  MOD_RES 23: note = when Xaa at position 23 is K, then K is chemically modified by conjugation of the epsilon-amino group of the K side chain with K(2-[2-(2-amino-ethoxy)-ethoxy]-acetyl)2-(gamma-Glu)-CO-(CH2)q-CO 2H
  VARIANT 24: note = Xaa at position 24 is selected from the group consisting of S, Aad, D-Glu, E, Aib, H, V, A, Q, D, P, and K
  MOD_RES 24: note = when Xaa at position 24 is K, then K is chemically modified by conjugation of the epsilon-amino group of the K side chain with K(2-[2-(2-amino-ethoxy)-ethoxy]-acetyl)2-(gamma-Glu)-CO-(CH2)q-CO 2H
  VARIANT 25: note = Xaa at position 25 is selected from the group consisting of Y or alpha-MeY
  VARIANT 26: note = Xaa at position 26 is selected from the group consisting of L, alpha-MeL, and K
  MOD_RES 26: note = when Xaa at position 26 is K, then K is chemically modified by conjugation of the epsilon-amino group of the K side chain with (2-[2-(2-amino-ethoxy)-ethoxy]-acetyl)2-(gamma-Glu)-CO-(CH2)q-CO2 H
  VARIANT 27: note = Xaa at position 27 is selected from the group consisting of L, I, and K
  MOD_RES 27: note = when Xaa at position 27 is K, then K is chemically modified by conjugation of the epsilon-amino group of the K side chain with (2-[2-(2-amino-ethoxy)-ethoxy]-acetyl)2-(gamma-Glu)-CO-(CH2)q-CO2 H
  VARIANT 28: note = Xaa at position 28 is selected from the group consisting of E, A, S, D-Glu, and K
  MOD_RES 28: note = when Xaa at position 28 is K, then K is chemically modified by conjugation of the epsilon-amino group of the K side chain with (2-[2-(2-amino-ethoxy)-ethoxy]-acetyl)2-(gamma-Glu)-CO-(CH2)q-CO2 H
  VARIANT 29: note = Xaa at position 29 is selected from the group consisting of Aib, G, A, and K
  MOD_RES 29: note = when Xaa at position 29 is K, then K is chemically modified by conjugation of the epsilon-amino group of the K side chain with (2-[2-(2-amino-ethoxy)-ethoxy]-acetyl)2-(gamma-Glu)-CO-(CH2)q-CO2 H
  VARIANT 30: note = Xaa at position 30 is selected from the group consisting of C, G, G-R2, and K, wherein R2 is a modification of the C-terminal group, wherein the modification is NH2 or absent, wherein if X30 is G-R2, then X31 is absent.
  MOD_RES 30: note = when Xaa at position 30 is K, then K is chemically modified by conjugation of the epsilon-amino group of the K side chain with (2-[2-(2-amino-ethoxy)-ethoxy]-acetyl)2-(gamma-Glu)-CO-(CH2)q-CO2 H
  VARIANT 31: note = Xaa at position 31 is absent or is selected from the group consisting of SEQ ID NO:4, SEQ ID NO:5, SEQ ID:6, SEQ ID NO:7, SEQ ID NO:8, and SEQ ID NO:9
  SITE 31: note = MISC_FEATURE - wherein no more than one of X10, X12, X13, X14, X16, X17, X19, X20, X21, X23, X24, X26, X27, X28, X29, X30, X31, X32, X33, X34, X35, X36, X37, X38, X39, and X40 may be a substituent that contains a fatty acid
  SITE 31: note = MISC_FEATURE - wherein no more than one of X30, X34, X39, and X40 may be C
  SITE 31: note = MISC_FEATURE - wherein if one of X30, X34, X39, and X40 is C, then none of X10, X12, X13, X14, X16, X17, X19, X20, X21, X23, X24, X26, X27, X28, X29, X30, X31, X32, X33, X34, X35, X36, X37, X38, X39, and X40 is a substituent that contains a fatty acid
  MOD_RES 31: note = Xaa at position 31 is modified with R2, wherein the modification is NH2 to form a C-terminal amide or absent
XXXGTXTSDXXXXXDXXAXXXXXXXXXXXXX

SEQ ID NO: 4-9 - skipped (6 entries)

SEQ ID NO: 10 - protein, 39 aa, synthetic construct
  REGION 1..39: note = Synthetic Construct
  SITE 2: note = MISC_FEATURE - Xaa at position 2 is Aib
  SITE 6: note = MISC_FEATURE - Xaa at position 6 is alpha-MeF(2F)
  SITE 13: note = MISC_FEATURE - Xaa at position 13 is alpha-MeL
  MOD_RES 17: note = K at position 17 is chemically modified by conjugation of the epsilon-amino group of the K side chain with (2-[2-(2-amino-ethoxy)-ethoxy]-acetyl)2-(gamma-Glu)-CO-(CH2)18-CO2H
  SITE 20: note = MISC_FEATURE - Xaa at position 20 is Aib
  SITE 24: note = MISC_FEATURE - Xaa at position 24 is D-Glu
  MOD_RES 39: note = The Serine at position 39 is amidated
YXEGTXTSDYSIXLDEKAQXEFIXYLIEGGPSSGAPPPS

SEQ ID NO: 11 - protein, 39 aa, synthetic construct
  REGION 1..39: note = Synthetic Construct
  SITE 2: note = MISC_FEATURE - Xaa at position 2 is Aib
  SITE 6: note = MISC_FEATURE - Xaa at position 6 is alpha-MeF(2F)
  SITE 13: note = MISC_FEATURE - Xaa at position 13 is alpha-MeL
  SITE 16: note = MISC_FEATURE - Xaa at position 16 is Orn
  MOD_RES 17: note = K at position 17 is chemically modified by conjugation of the epsilon-amino group of the K side chain with (2-[2-(2-amino-ethoxy)-ethoxy]-acetyl)2-(gamma-Glu)-CO-(CH2)16-CO2H
  SITE 20: note = MISC_FEATURE - Xaa at position 20 is Aib
  SITE 24: note = MISC_FEATURE - Xaa at position 24 is D-Glu
  MOD_RES 39: note = The Serine at position 39 is amidated
YXEGTXTSDYSIXLDXKAQXEFIXYLIEGGPSSGAPPPS

SEQ ID NO: 12 - protein, 39 aa, synthetic construct; identical to SEQ ID NO: 11
  REGION 1..39: note = Synthetic Construct
  SITE 2: note = MISC_FEATURE - Xaa at position 2 is Aib
  SITE 6: note = MISC_FEATURE - Xaa at position 6 is alpha-MeF(2F)
  SITE 13: note = MISC_FEATURE - Xaa at position 13 is alpha-MeL
  SITE 16: note = MISC_FEATURE - Xaa at position 16 is Orn
  MOD_RES 17: note = K at position 17 is chemically modified by conjugation of the epsilon-amino group of the K side chain with (2-[2-(2-amino-ethoxy)-ethoxy]-acetyl)2-(gamma-Glu)-CO-(CH2)18-CO 2H
  SITE 20: note = MISC_FEATURE - Xaa at position 20 is Aib
  SITE 24: note = MISC_FEATURE - Xaa at position 24 is D-Glu
  SITE 39: note = MISC_FEATURE - The Serine at position 39 is amidated

SEQ ID NO: 13 - protein, 39 aa, synthetic construct
  REGION 1..39: note = Synthetic Construct
  SITE 2: note = MISC_FEATURE - Xaa at position 2 is Aib
  SITE 6: note = MISC_FEATURE - Xaa at position 6 is alpha-MeF(2F)
  SITE 10: note = MISC_FEATURE - Xaa at position 10 is 4Pal
  SITE 13: note = MISC_FEATURE - Xaa at position 13 is alpha-MeL
  SITE 16: note = MISC_FEATURE - Xaa at position 16 is Orn
  MOD_RES 17: note = K at position 17 is chemically modified by conjugation of the epsilon-amino group of the K side chain with (2-[2-(2-amino-ethoxy)-ethoxy]-acetyl)2-(gamma-Glu)-CO-(CH2)16-CO 2H
  SITE 20: note = MISC_FEATURE - Xaa at position 20 is Aib
  SITE 24: note = MISC_FEATURE - Xaa at position 24 is D-Glu
  SITE 25: note = MISC_FEATURE - Xaa at position 25 is alpha-MeY
  MOD_RES 39: note = The Serine at position 39 is amidated
YXEGTXTSDXSIXLDXKAQXEFIXXLIEGGPSSGAPPPS

SEQ ID NO: 14 - protein, 39 aa, synthetic construct
  REGION 1..39: note = Synthetic Construct
  SITE 2: note = MISC_FEATURE - Xaa at position 2 is Aib
  MOD_RES 17: note = Lys at position 17 is chemically modified by conjugation of the epsilon-amino group of the Lys side chain with (2-[2-(2-amino-ethoxy)-ethoxy]-acetyl)2-(gamma-Glu)-CO-(CH2)18-CO 2H
  SITE 20: note = MISC_FEATURE - Xaa at position 20 is Aib
  MOD_RES 39: note = Ser at position 39 is amidated
YXEGTFTSDYSILLDKKAQXAFIEYLIEGGPSSGAPPPS

SEQ ID NO: 15 - protein, 39 aa, synthetic construct
  REGION 1..39: note = Synthetic Construct
  SITE 2: note = MISC_FEATURE - Xaa at position 2 is Aib
  MOD_RES 17: note = Lys at position 17 is chemically modified by conjugation of the epsilon-amino group of the Lys side chain with (2-[2-(2-amino-ethoxy)-ethoxy]-acetyl)2-(gamma-Glu)-CO-(CH2)18-CO 2H
  SITE 20: note = MISC_FEATURE - Xaa at position 20 is Aib
  MOD_RES 39: note = Ser at position 39 is amidated
YXEGTFTSDYSILLDSKAQXAFIEYLIEGGPSSGAPPPS

SEQ ID NO: 16 - protein, 39 aa, synthetic construct
  REGION 1..39: note = Synthetic Construct
  SITE 2: note = MISC_FEATURE - Xaa at position 2 is Aib
  SITE 13: note = MISC_FEATURE - Xaa at position 13 is alpha-methyl-Leu
  MOD_RES 17: note = Lys at position 17 is chemically modified by conjugation of the epsilon-amino group of the Lys side chain with (2-[2-(2-amino-ethoxy)-ethoxy]-acetyl)2-(gamma-Glu)-CO-(CH2)18-CO 2H
  SITE 20: note = MISC_FEATURE - Xaa at position 20 is Aib
  MOD_RES 39: note = Ser at position 39 is amidated
YXEGTFTSDYSIXLDKKAQXAFIEYLIEGGPSSGAPPPS

SEQ ID NO: 17 - protein, 39 aa, synthetic construct
  REGION 1..39: note = Synthetic Construct
  SITE 2: note = MISC_FEATURE - Xaa at position 2 is Aib
  SITE 13: note = MISC_FEATURE - Xaa at position 13 is alpha-methyl-Leu
  MOD_RES 17: note = Lys at position 17 is chemically modified by conjugation of the epsilon-amino group of the Lys side chain with (2-[2-(2-amino-ethoxy)-ethoxy]-acetyl)2-(gamma-Glu)-CO-(CH2)18-CO 2H
  SITE 20: note = MISC_FEATURE - Xaa at position 20 is alpha-methyl-Lys
  MOD_RES 39: note = Ser at position 39 is amidated
YXEGTFTSDYSIXLDEKAQXAFIEYLLEGGPSSGAPPPS

SEQ ID NO: 18 - protein, 39 aa, synthetic construct
  REGION 1..39: note = Synthetic Construct
  SITE 2: note = MISC_FEATURE - Xaa at position 2 is Aib
  SITE 13: note = MISC_FEATURE - Xaa at position 13 is alpha-methyl-Leu
  MOD_RES 17: note = Lys at position 17 is chemically modified by conjugation of the epsilon-amino group of the Lys side chain with (2-[2-(2-amino-ethoxy)-ethoxy]-acetyl)2-(gamma-Glu)-CO-(CH2)18-CO 2H
  SITE 20: note = MISC_FEATURE - Xaa at position 20 is alpha-methyl-Lys
  SITE 29: note = MISC_FEATURE - Xaa at position 29 is Aib
  MOD_RES 39: note = Ser at position 39 is amidated
YXEGTFTSDYSIXLDEKAQXAFIEYLLEXGPSSGAPPPS

SEQ ID NO: 19 - protein, 39 aa, synthetic construct
  REGION 1..39: note = Synthetic Construct
  SITE 2: note = MISC_FEATURE - Xaa at position 2 is Aib
  MOD_RES 12: note = Lys at position 12 is chemically modified by conjugation of the epsilon-amino group of the Lys side chain with (2-[2-(2-amino-ethoxy)-ethoxy]-acetyl)2-(gamma-Glu)-CO-(CH2)18-CO 2H
  SITE 20: note = MISC_FEATURE - Xaa at position 20 is Aib
  MOD_RES 39: note = Ser at position 39 is amidated
YXEGTFTSDYSKLLDKIAQXAFIEYLIEGGPSSGAPPPS

SEQ ID NO: 20 - protein, 39 aa, synthetic construct
  REGION 1..39: note = Synthetic Construct
  SITE 2: note = MISC_FEATURE - Xaa at position 2 is Aib
  MOD_RES 13: note = Lys at position 13 is chemically modified by conjugation of the epsilon-amino group of the Lys side chain with (2-[2-(2-amino-ethoxy)-ethoxy]-acetyl)2-(gamma-Glu)-CO-(CH2)18-CO 2H
  SITE 20: note = MISC_FEATURE - Xaa at position 20 is Aib
  MOD_RES 39: note = Ser at position 39 is amidated
YXEGTFTSDYSIKLDKIAQXAFIEYLIEGGPSSGAPPPS

SEQ ID NO: 21 - protein, 39 aa, synthetic construct
  REGION 1..39: note = Synthetic Construct
  SITE 2: note = MISC_FEATURE - Xaa at position 2 is Aib
  MOD_RES 16: note = Lys at position 16 is chemically modified by conjugation of the epsilon-amino group of the Lys side chain with (2-[2-(2-amino-ethoxy)-ethoxy]-acetyl)2-(gamma-Glu)-CO-(CH2)18-CO 2H
  SITE 20: note = MISC_FEATURE - Xaa at position 20 is Aib
  MOD_RES 39: note = Ser at position 39 is amidated
YXEGTFTSDYSILLDKIAQXAFIEYLIEGGPSSGAPPPS

SEQ ID NO: 22 - protein, 39 aa, synthetic construct
  REGION 1..39: note = Synthetic Construct
  SITE 2: note = MISC_FEATURE - Xaa at position 2 is Aib
  MOD_RES 19: note = Lys at position 19 is chemically modified by conjugation of the epsilon-amino group of the Lys side chain with (2-[2-(2-amino-ethoxy)-ethoxy]-acetyl)2-(gamma-Glu)-CO-(CH2)18-CO 2H
  SITE 20: note = MISC_FEATURE - Xaa at position 20 is Aib
  MOD_RES 39: note = Ser at position 39 is amidated
YXEGTFTSDYSILLDKIAKXAFIEYLIEGGPSSGAPPPS

SEQ ID NO: 23 - protein, 39 aa, synthetic construct
  REGION 1..39: note = Synthetic Construct
  SITE 2: note = MISC_FEATURE - Xaa at position 2 is Aib
  SITE 20: note = MISC_FEATURE - Xaa at position 20 is Aib
  MOD_RES 21: note = Lys at position 17 is chemically modified by conjugation of the epsilon-amino group of the Lys side chain with (2-[2-(2-amino-ethoxy)-ethoxy]-acetyl)2-(gamma-Glu)-CO-(CH2)18-CO 2H
  MOD_RES 39: note = Ser at position 39 is amidated
YXEGTFTSDYSILLDKIAQXKFIEYLIEGGPSSGAPPPS

SEQ ID NO: 24 - protein, 39 aa, synthetic construct
  REGION 1..39: note = Synthetic Construct
  SITE 2: note = MISC_FEATURE - Xaa at position 2 is Aib
  SITE 20: note = MISC_FEATURE - Xaa at position 20 is Aib
  MOD_RES 23: note = Lys at position 23 is chemically modified by conjugation of the epsilon-amino group of the Lys side chain with (2-[2-(2-amino-ethoxy)-ethoxy]-acetyl)2-(gamma-Glu)-CO-(CH2)18-CO 2H
  MOD_RES 39: note = Ser at position 39 is amidated
YXEGTFTSDYSILLDKIAQXAFKEYLIEGGPSSGAPPPS

SEQ ID NO: 25 - protein, 39 aa, synthetic construct
  REGION 1..39: note = Synthetic Construct
  SITE 2: note = MISC_FEATURE - Xaa at position 2 is Aib
  SITE 20: note = MISC_FEATURE - Xaa at position 20 is Aib
  MOD_RES 24: note = Lys at position 24 is chemically modified by conjugation of the epsilon-amino group of the Lys side chain with (2-[2-(2-amino-ethoxy)-ethoxy]-acetyl)2-(gamma-Glu)-CO-(CH2)18-CO 2H
  MOD_RES 39: note = Ser at position 39 is amidated
YXEGTFTSDYSILLDKIAQXAFIKYLIEGGPSSGAPPPS

SEQ ID NO: 26 - protein, 39 aa, synthetic construct
  REGION 1..39: note = Synthetic Construct
  SITE 2: note = MISC_FEATURE - Xaa at position 2 is Aib
  SITE 20: note = MISC_FEATURE - Xaa at position 20 is Aib
  MOD_RES 28: note = Lys at position 28 is chemically modified by conjugation of the epsilon-amino group of the Lys side chain with (2-[2-(2-amino-ethoxy)-ethoxy]-acetyl)2-(gamma-Glu)-CO-(CH2)18-CO 2H
  MOD_RES 39: note = Ser at position 39 is amidated
YXEGTFTSDYSILLDKIAQXAFIEYLIKGGPSSGAPPPS

SEQ ID NO: 27 - protein, 39 aa, synthetic construct
  REGION 1..39: note = Synthetic Construct
  SITE 2: note = MISC_FEATURE - Xaa at position 2 is Aib
  SITE 20: note = MISC_FEATURE - Xaa at position 20 is Aib
  MOD_RES 32: note = Lys at position 32 is chemically modified by conjugation of the epsilon-amino group of the Lys side chain with (2-[2-(2-amino-ethoxy)-ethoxy]-acetyl)2-(gamma-Glu)-CO-(CH2)18-CO 2H
  MOD_RES 39: note = Ser at position 39 is amidated
YXEGTFTSDYSILLDKIAQXAFIEYLIEGGPKSGAPPPS

SEQ ID NO: 28 - protein, 39 aa, synthetic construct
  REGION 1..39: note = Synthetic Construct
  SITE 2: note = MISC_FEATURE - Xaa at position 2 is Aib
  SITE 20: note = MISC_FEATURE - Xaa at position 20 is Aib
  MOD_RES 37: note = Lys at position 37 is chemically modified by conjugation of the epsilon-amino group of the Lys side chain with (2-[2-(2-amino-ethoxy)-ethoxy]-acetyl)2-(gamma-Glu)-CO-(CH2)18-CO 2H
  MOD_RES 39: note = Ser at position 39 is amidated
YXEGTFTSDYSILLDKIAQXAFIEYLIEGGPSSGAPKPS

SEQ ID NO: 29 - protein, 39 aa, synthetic construct
  REGION 1..39: note = Synthetic Construct
  SITE 2: note = MISC_FEATURE - Xaa at position 2 is Aib
  SITE 20: note = MISC_FEATURE - Xaa at position 20 is Aib
  MOD_RES 38: note = Lys at position 38 is chemically modified by conjugation of the epsilon-amino group of the Lys side chain with (2-[2-(2-amino-ethoxy)-ethoxy]-acetyl)2-(gamma-Glu)-CO-(CH2)18-CO 2H
  MOD_RES 39: note = Ser at position 39 is amidated
YXEGTFTSDYSILLDKIAQXAFIEYLIEGGPSSGAPPKS

SEQ ID NO: 30 - protein, 39 aa, synthetic construct
  REGION 1..39: note = Synthetic Construct
  SITE 2: note = MISC_FEATURE - Xaa at position 2 is Aib
  SITE 20: note = MISC_FEATURE - Xaa at position 20 is Aib
  MOD_RES 39: note = Lys at position 39 is chemically modified by conjugation of the epsilon-amino group of the Lys side chain with (2-[2-(2-amino-ethoxy)-ethoxy]-acetyl)2-(gamma-Glu)-CO-(CH2)18-CO 2H
  MOD_RES 39: note = Lys at position 39 is amidated
YXEGTFTSDYSILLDKIAQXAFIEYLIEGGPSSGAPPPK

SEQ ID NO: 31 - protein, 34 aa, synthetic construct
  REGION 1..34: note = Synthetic Construct
  SITE 2: note = MISC_FEATURE - Xaa at position 2 is Aib
  MOD_RES 17: note = Lys at position 17 is chemically modified by conjugation of the epsilon-amino group of the Lys side chain with (2-[2-(2-amino-ethoxy)-ethoxy]-acetyl)2-(gamma-Glu)-CO-(CH2)18-CO 2H
  SITE 20: note = MISC_FEATURE - Xaa at position 20 is Aib
  MOD_RES 34: note = Gly at position 34 is amidated
YXEGTFTSDYSILLDKKAQXAFIEYLIEGGPSSG

SEQ ID NO: 32 - protein, 30 aa, synthetic construct
  REGION 1..30: note = Synthetic Construct
  SITE 2: note = MISC_FEATURE - Xaa at position 2 is Aib
  MOD_RES 17: note = Lys at position 17 is chemically modified by conjugation of the epsilon-amino group of the Lys side chain with (2-[2-(2-amino-ethoxy)-ethoxy]-acetyl)2-(gamma-Glu)-CO-(CH2)18-CO 2H
  SITE 20: note = MISC_FEATURE - Xaa at position 20 is Aib
  MOD_RES 30: note = Gly at position 30 is amidated
YXEGTFTSDYSILLDKKAQXAFIEYLIEGG

SEQ ID NO: 33 - protein, 39 aa, synthetic construct
  REGION 1..39: note = Synthetic Construct
  SITE 2: note = MISC_FEATURE - Xaa at position 2 is Aib
  SITE 13: note = MISC_FEATURE - Xaa at position 13 is alpha-methyl-Leu
  MOD_RES 17: note = Lys at position 17 is chemically modified by conjugation of the epsilon-amino group of the Lys side chain with (2-[2-(2-amino-ethoxy)-ethoxy]-acetyl)2-(gamma-Glu)-CO-(CH2)18-CO 2H
  SITE 20: note = MISC_FEATURE - Xaa at position 20 is Aib
  MOD_RES 39: note = Ser at position 39 is amidated
YXEGTFTSDYSIXLDSKAQXAFIEYLIEGGPSSGAPPPS

SEQ ID NO: 34 - protein, 39 aa, synthetic construct
  REGION 1..39: note = Synthetic Construct
  SITE 2: note = MISC_FEATURE - Xaa at position 2 is Aib
  SITE 13: note = MISC_FEATURE - Xaa at position 13 is alpha-methyl-Leu
  SITE 16: note = MISC_FEATURE - Xaa at position 16 is Aib
  MOD_RES 17: note = Lys at position 17 is chemically modified by conjugation of the epsilon-amino group of the Lys side chain with (2-[2-(2-amino-ethoxy)-ethoxy]-acetyl)2-(gamma-Glu)-CO-(CH2)18-CO 2H
  SITE 20: note = MISC_FEATURE - Xaa at position 20 is Aib
  MOD_RES 39: note = Ser at position 39 is amidated
YXEGTFTSDYSIXLDXKAQXAFIEYLIEGGPSSGAPPPS

SEQ ID NO: 35 - protein, 30 aa, synthetic construct
  REGION 1..30: note = Synthetic Construct
  SITE 2: note = MISC_FEATURE - Xaa at position 2 is Aib
  SITE 13: note = MISC_FEATURE - Xaa at position 13 is alpha-methyl-Leu
  MOD_RES 17: note = Lys at position 17 is chemically modified by conjugation of the epsilon-amino group of the Lys side chain with (2-[2-(2-amino-ethoxy)-ethoxy]-acetyl)2-(gamma-Glu)-CO-(CH2)18-CO 2H
  SITE 20: note = MISC_FEATURE - Xaa at position 20 is Aib
  MOD_RES 30: note = Gly at position 30 is amidated
YXEGTFTSDYSIXLDKKAQXAFIEYLIEGG

SEQ ID NO: 36 - protein, 30 aa, synthetic construct
  REGION 1..30: note = Synthetic Construct
  SITE 2: note = MISC_FEATURE - Xaa at position 2 is Aib
  SITE 13: note = MISC_FEATURE - Xaa at position 13 is alpha-methyl-Leu
  MOD_RES 17: note = Lys at position 17 is chemically modified by conjugation of the epsilon-amino group of the Lys side chain with (2-[2-(2-amino-ethoxy)-ethoxy]-acetyl)2-(gamma-Glu)-CO-(CH2)18-CO 2H
  SITE 20: note = MISC_FEATURE - Xaa at position 20 is Aib
  MOD_RES 30: note = Gly at position 30 is amidated
YXEGTFTSDYSIXLDEKAQXAFIEYLIEGG

SEQ ID NO: 37 - protein, 30 aa, synthetic construct
  REGION 1..30: note = Synthetic Construct
  SITE 2: note = MISC_FEATURE - Xaa at position 2 is Aib
  SITE 13: note = MISC_FEATURE - Xaa at position 13 is alpha-methyl-Leu
  MOD_RES 17: note = Lys at position 17 is chemically modified by conjugation of the epsilon-amino group of the Lys side chain with (2-[2-(2-amino-ethoxy)-ethoxy]-acetyl)2-(gamma-Glu)-CO-(CH2)18-CO 2H
  SITE 20: note = MISC_FEATURE - Xaa at position 20 is Aib
  MOD_RES 30: note = Gly at position 30 is amidated
YXEGTFTSDYSIXLDSKAQXAFIEYLIEGG

SEQ ID NO: 38 - protein, 30 aa, synthetic construct
  REGION 1..30: note = Synthetic Construct
  SITE 2: note = MISC_FEATURE - Xaa at position 2 is Aib
  SITE 13: note = MISC_FEATURE - Xaa at position 13 is alpha-methyl-Leu
  MOD_RES 17: note = Lys at position 17 is chemically modified by conjugation of the epsilon-amino group of the Lys side chain with (2-[2-(2-amino-ethoxy)-ethoxy]-acetyl)2-(gamma-Glu)-CO-(CH2)18-CO 2H
  SITE 20: note = MISC_FEATURE - Xaa at position 20 is Aib
  MOD_RES 30: note = Gly at position 30 is amidated
YXEGTFTSDYSIXLDTKAQXAFIEYLIEGG

SEQ ID NO: 39 - protein, 39 aa, synthetic construct; identical to SEQ ID NO: 17
  REGION 1..39: note = Synthetic Construct
  SITE 2: note = MISC_FEATURE - Xaa at position 2 is Aib
  SITE 13: note = MISC_FEATURE - Xaa at position 13 is alpha-methyl-Leu
  MOD_RES 17: note = Lys at position 17 is chemically modified by conjugation of the epsilon-amino group of the Lys side chain with (2-[2-(2-amino-ethoxy)-ethoxy]-acetyl)2-(gamma-Glu)-CO-(CH2)18-CO 2H
  SITE 20: note = MISC_FEATURE - Xaa at position 20 is Aib
  MOD_RES 39: note = Ser at position 39 is amidated

SEQ ID NO: 40 - protein, 39 aa, synthetic construct
  REGION 1..39: note = Synthetic Construct
  SITE 2: note = MISC_FEATURE - Xaa at position 2 is Aib
  SITE 11: note = MISC_FEATURE - Xaa at position 11 is alpha-methyl-Ser
  MOD_RES 17: note = Lys at position 17 is chemically modified by conjugation of the epsilon-amino group of the Lys side chain with (2-[2-(2-amino-ethoxy)-ethoxy]-acetyl)2-(gamma-Glu)-CO-(CH2)18-CO 2H
  SITE 20: note = MISC_FEATURE - Xaa at position 20 is Aib
  MOD_RES 39: note = Ser at position 39 is amidated
YXEGTFTSDYXILLDKKAQXAFIEYLIEGGPSSGAPPPS

SEQ ID NO: 41 - protein, 39 aa, synthetic construct
  REGION 1..39: note = Synthetic Construct
  SITE 2: note = MISC_FEATURE - Xaa at position 2 is Aib
  SITE 6: note = MISC_FEATURE - Xaa at position 6 is alpha-methyl-Phe
  SITE 13: note = MISC_FEATURE - Xaa at position 13 is alpha-methyl-Leu
  MOD_RES 17: note = Lys at position 17 is chemically modified by conjugation of the epsilon-amino group of the Lys side chain with (2-[2-(2-amino-ethoxy)-ethoxy]-acetyl)2-(gamma-Glu)-CO-(CH2)18-CO 2H
  SITE 20: note = MISC_FEATURE - Xaa at position 20 is Aib
  MOD_RES 39: note = Ser at position 39 is amidated
YXEGTXTSDYSIXLDKKAQXAFIEYLIEGGPSSGAPPPS

SEQ ID NO: 42 - protein, 30 aa, synthetic construct
  REGION 1..30: note = Synthetic Construct
  SITE 2: note = MISC_FEATURE - Xaa at position 2 is Aib
  SITE 20: note = MISC_FEATURE - Xaa at position 20 is Aib
  MOD_RES 28: note = Lys at position 28 is chemically modified by conjugation of the epsilon-amino group of the Lys side chain with (2-[2-(2-amino-ethoxy)-ethoxy]-acetyl)2-(gamma-Glu)-CO-(CH2)18-CO 2H
  MOD_RES 30: note = Gly at position 30 is amidated
YXEGTFTSDYSILLDKIAQXAFIEYLIKGG

SEQ ID NO: 43 - protein, 39 aa, synthetic construct; identical to SEQ ID NO: 14
  REGION 1..39: note = Synthetic Construct
  SITE 2: note = MISC_FEATURE - Xaa at position 2 is D-Ala
  MOD_RES 17: note = Lys at position 17 is chemically modified by conjugation of the epsilon-amino group of the Lys side chain with (2-[2-(2-amino-ethoxy)-ethoxy]-acetyl)2-(gamma-Glu)-CO-(CH2)18-CO 2H
  SITE 20: note = MISC_FEATURE - Xaa at position 20 is Aib
  MOD_RES 39: note = Ser at position 39 is amidated

SEQ ID NO: 44 - protein, 39 aa, synthetic construct; identical to SEQ ID NO: 40
  REGION 1..39: note = Synthetic Construct
  SITE 2: note = MISC_FEATURE - Xaa at position 2 is Aib
  SITE 11: note = MISC_FEATURE - Xaa at position 11 is D-Ser
  MOD_RES 17: note = Lys at position 17 is chemically modified by conjugation of the epsilon-amino group of the Lys side chain with (2-[2-(2-amino-ethoxy)-ethoxy]-acetyl)2-(gamma-Glu)-CO-(CH2)18-CO 2H
  SITE 20: note = MISC_FEATURE - Xaa at position 20 is Aib
  MOD_RES 39: note = Ser at position 39 is amidated

SEQ ID NO: 45 - protein, 39 aa, synthetic construct
  REGION 1..39: note = Synthetic Construct
  SITE 2: note = MISC_FEATURE - Xaa at position 2 is Aib
  MOD_RES 17: note = Lys at position 17 is chemically modified by conjugation of the epsilon-amino group of the Lys side chain with (2-[2-(2-amino-ethoxy)-ethoxy]-acetyl)2-(gamma-Glu)-CO-(CH2)18-CO 2H
  SITE 20: note = MISC_FEATURE - Xaa at position 20 is Aib
  SITE 28: note = MISC_FEATURE - Xaa at position 28 is D-Glu
  MOD_RES 39: note = Ser at position 39 is amidated
YXEGTFTSDYSILLDKKAQXAFIEYLIXGGPSSGAPPPS

SEQ ID NO: 46 - protein, 39 aa, synthetic construct
  REGION 1..39: note = Synthetic Construct
  SITE 2: note = MISC_FEATURE - Xaa at position 2 is Aib
  MOD_RES 17: note = Lys at position 17 is chemically modified by conjugation of the epsilon-amino group of the Lys side chain with (2-[2-(2-amino-ethoxy)-ethoxy]-acetyl)2-(gamma-Glu)-CO-(CH2)18-CO 2H
  SITE 20: note = MISC_FEATURE - Xaa at position 20 is Aib
  SITE 24: note = MISC_FEATURE - Xaa at position 24 is D-Glu
  MOD_RES 39: note = Ser at position 39 is amidated
YXEGTFTSDYSILLDKKAQXAFIXYLIEGGPSSGAPPPS

SEQ ID NO: 47 - protein, 39 aa, synthetic construct
  REGION 1..39: note = Synthetic Construct
  MOD_RES 17: note = Lys at position 17 is chemically modified by conjugation of the epsilon-amino group of the Lys side chain with (2-[2-(2-amino-ethoxy)-ethoxy]-acetyl)2-(gamma-Glu)-CO-(CH2)18-CO 2H
  SITE 20: note = MISC_FEATURE - Xaa at position 20 is Aib
  MOD_RES 39: note = Ser at position 39 is amidated
YPEGTFTSDYSILLDKKAQXAFIEYLIEGGPSSGAPPPS

SEQ ID NO: 48 - protein, 39 aa, synthetic construct
  REGION 1..39: note = Synthetic Construct
  SITE 2: note = MISC_FEATURE - Xaa at position 2 is Aib
  SITE 3: note = MISC_FEATURE - Xaa at position 3 is Aad
  MOD_RES 17: note = Lys at position 17 is chemically modified by conjugation of the epsilon-amino group of the Lys side chain with (2-[2-(2-amino-ethoxy)-ethoxy]-acetyl)2-(gamma-Glu)-CO-(CH2)18-CO 2H
  SITE 20: note = MISC_FEATURE - Xaa at position 20 is Aib
  MOD_RES 39: note = Ser at position 39 is amidated
YXXGTFTSDYSILLDKKAQXAFIEYLIEGGPSSGAPPPS

SEQ ID NO: 49 - protein, 30 aa, synthetic construct
  REGION 1..30: note = Synthetic Construct
  SITE 2: note = MISC_FEATURE - Xaa at position 2 is Aib
  SITE 6: note = MISC_FEATURE - Xaa at position 6 is alpha-methyl-Phe
  SITE 20: note = MISC_FEATURE - Xaa at position 20 is Aib
  MOD_RES 28: note = Lys at position 28 is chemically modified by conjugation of the epsilon-amino group of the Lys side chain with (2-[2-(2-amino-ethoxy)-ethoxy]-acetyl)2-(gamma-Glu)-CO-(CH2)18-CO 2H
  MOD_RES 30: note = Gly at position 30 is amidated
YXEGTXTSDYSILLDKIAQXAFIEYLIKGG

SEQ ID NO: 50 - protein, 30 aa, synthetic construct
  REGION 1..30: note = Synthetic Construct
  SITE 2: note = MISC_FEATURE - Xaa at position 2 is Aib
  SITE 13: note = MISC_FEATURE - Xaa at position 13 is alpha-methyl-Leu
  SITE 20: note = MISC_FEATURE - Xaa at position 20 is Aib
  MOD_RES 28: note = Lys at position 28 is chemically modified by conjugation of the epsilon-amino group of the Lys side chain with (2-[2-(2-amino-ethoxy)-ethoxy]-acetyl)2-(gamma-Glu)-CO-(CH2)18-CO 2H
  MOD_RES 30: note = Gly at position 30 is amidated
YXEGTFTSDYSIXLDKIAQXAFIEYLIKGG

SEQ ID NO: 51 - protein, 30 aa, synthetic construct
  REGION 1..30: note = Synthetic Construct
  SITE 2: note = MISC_FEATURE - Xaa at position 2 is Aib
  SITE 6: note = MISC_FEATURE - Xaa at position 13 is alpha-methyl-Phe
  MOD_RES 17: note = Lys at position 17 is chemically modified by conjugation of the epsilon-amino group of the Lys side chain with (2-[2-(2-amino-ethoxy)-ethoxy]-acetyl)2-(gamma-Glu)-CO-(CH2)18-CO 2H
  SITE 20: note = MISC_FEATURE - Xaa at position 20 is Aib
  MOD_RES 30: note = Gly at position 30 is amidated
YXEGTXTSDYSILLDKKAQXAFIEYLIEGG

SEQ ID NO: 52 - protein, 30 aa, synthetic construct
  REGION 1..30: note = Synthetic Construct
  SITE 2: note = MISC_FEATURE - Xaa at position 2 is Aib
  SITE 6: note = MISC_FEATURE - Xaa at position 6 is alpha-methyl-Phe
  SITE 13: note = MISC_FEATURE - Xaa at position 13 is alpha-methyl-Leu
  MOD_RES 17: note = Lys at position 17 is chemically modified by conjugation of the epsilon-amino group of the Lys side chain with (2-[2-(2-amino-ethoxy)-ethoxy]-acetyl)2-(gamma-Glu)-CO-(CH2)18-CO 2H
  SITE 20: note = MISC_FEATURE - Xaa at position 20 is Aib
  MOD_RES 30: note = Gly at position 30 is amidated
YXEGTXTSDYSIXLDKKAQXAFIEYLIEGG

SEQ ID NO: 53 - protein, 30 aa, synthetic construct
  REGION 1..30: note = Synthetic Construct
  SITE 2: note = MISC_FEATURE - Xaa at position 2 is Aib
  SITE 6: note = MISC_FEATURE - Xaa at position 6 is alpha-methyl-Phe(2F)
  SITE 13: note = MISC_FEATURE - Xaa at position 13 is alpha-methyl-Leu
  MOD_RES 17: note = Lys at position 17 is chemically modified by conjugation of the epsilon-amino group of the Lys side chain with (2-[2-(2-amino-ethoxy)-ethoxy]-acetyl)2-(gamma-Glu)-CO-(CH2)18-CO 2H
  SITE 20: note = MISC_FEATURE - Xaa at position 20 is Aib
  MOD_RES 30: note = Gly at position 30 is amidated
YXEGTXTSDYSIXLDEKAQXEFIEYLIEGG

SEQ ID NO: 54 - protein, 30 aa, synthetic construct; identical to SEQ ID NO: 53
  REGION 1..30: note = Synthetic Construct
  SITE 2: note = MISC_FEATURE - Xaa at position 2 is Aib
  SITE 6: note = MISC_FEATURE - Xaa at position 6 is alpha-methyl-Phe(2F)
  SITE 13: note = MISC_FEATURE - Xaa at position 13 is alpha-methyl-Leu
  MOD_RES 17: note = Lys at position 17 is chemically modified by conjugation of the epsilon-amino group of the Lys side chain with (2-[2-(2-amino-ethoxy)-ethoxy]-acetyl)2-(gamma-Glu)-CO-(CH2)16-CO 2H
  SITE 20: note = MISC_FEATURE - Xaa at position 20 is Aib
  MOD_RES 30: note = Gly at position 30 is amidated

SEQ ID NO: 55 - protein, 39 aa, synthetic construct; identical to SEQ ID NO: 14
  REGION 1..39: note = Synthetic Construct
  SITE 2: note = MISC_FEATURE - Xaa at position 2 is Aib
  MOD_RES 17: note = Lys at position 17 is chemically modified by conjugation of the epsilon-amino group of the Lys side chain with (2-[2-(2-amino-ethoxy)-ethoxy]-acetyl)-AOC-(gamma-Glu)-CO-(CH2)18 -CO2H
  SITE 20: note = MISC_FEATURE - Xaa at position 20 is Aib
  MOD_RES 39: note = Ser at position 39 is amidated

SEQ ID NO: 56 - protein, 39 aa, synthetic construct; identical to SEQ ID NO: 14
  REGION 1..39: note = Synthetic Construct
  SITE 2: note = MISC_FEATURE - Xaa at position 2 is Aib
  MOD_RES 17: note = Lys at position 17 is chemically modified by conjugation of the epsilon-amino group of the Lys side chain with AOC-(2-[2-(2-amino-ethoxy)-ethoxy]-acetyl)-(gamma-Glu)-CO-(CH2)18 -CO2H
  SITE 20: note = MISC_FEATURE - Xaa at position 20 is Aib
  MOD_RES 39: note = Ser at position 39 is amidated

SEQ ID NO: 57 - protein, 39 aa, synthetic construct; identical to SEQ ID NO: 14
  REGION 1..39: note = Synthetic Construct
  SITE 2: note = MISC_FEATURE - Xaa at position 2 is Aib
  MOD_RES 17: note = Lys at position 17 is chemically modified by conjugation of the epsilon-amino group of the Lys side chain with (2-[2-(2-amino-ethoxy)-ethoxy]-acetyl)-(gamma-Glu)-(Trx)-CO-(CH2) 18-CO2H
  SITE 20: note = MISC_FEATURE - Xaa at position 20 is Aib
  MOD_RES 39: note = Ser at position 39 is amidated

SEQ ID NO: 58 - protein, 39 aa, synthetic construct; identical to SEQ ID NO: 14
  REGION 1..39: note = Synthetic Construct
  SITE 2: note = MISC_FEATURE - Xaa at position 2 is Aib
  MOD_RES 17: note = Lys at position 17 is chemically modified by conjugation of the epsilon-amino group of the Lys side chain with (2-[2-(2-amino-ethoxy)-ethoxy]-acetyl)-(Trx)-(gamma-Glu)-CO-(CH2) 18-CO2H
  SITE 20: note = MISC_FEATURE - Xaa at position 20 is Aib
  MOD_RES 39: note = Ser at position 39 is amidated

SEQ ID NO: 59 - protein, 39 aa, synthetic construct; identical to SEQ ID NO: 14
  REGION 1..39: note = Synthetic Construct
  SITE 2: note = MISC_FEATURE - Xaa at position 2 is Aib
  MOD_RES 17: note = Lys at position 17 is chemically modified by conjugation of the epsilon-amino group of the Lys side chain with (2-[2-(2-amino-ethoxy)-ethoxy]-acetyl)-(epsilon-Lys)-(gamma-Glu)- CO-(CH2)18-CO2H
  SITE 20: note = MISC_FEATURE - Xaa at position 20 is Aib
  MOD_RES 39: note = Ser at position 39 is amidated

SEQ ID NO: 60 - protein, 39 aa, synthetic construct; identical to SEQ ID NO: 14
  REGION 1..39: note = Synthetic Construct
  SITE 2: note = MISC_FEATURE - Xaa at position 2 is Aib
  MOD_RES 17: note = Lys at position 17 is chemically modified by conjugation of the epsilon-amino group of the Lys side chain with (2-[2-(2-amino-ethoxy)-ethoxy]-acetyl)2-(epsilon-Lys)-CO-(CH2)18- CO2H
  SITE 20: note = MISC_FEATURE - Xaa at position 20 is Aib
  MOD_RES 39: note = Ser at position 39 is amidated

SEQ ID NO: 61 - protein, 39 aa, synthetic construct; identical to SEQ ID NO: 14
  REGION 1..39: note = Synthetic Construct
  SITE 2: note = MISC_FEATURE - Xaa at position 2 is Aib
  MOD_RES 17: note = Lys at position 17 is chemically modified by conjugation of the epsilon-amino group of the Lys side chain with (2-[2-(2-amino-ethoxy)-ethoxy]-acetyl)-(epsilon-Lys)-(epsilon-Lys )-CO-(CH2)18-CO2H
  SITE 20: note = MISC_FEATURE - Xaa at position 2 is Aib
  MOD_RES 39: note = Ser at position 39 is amidated

SEQ ID NO: 62 - protein, 39 aa, synthetic construct
  REGION 1..39: note = Synthetic Construct
  SITE 2: note = MISC_FEATURE - Xaa at position 2 is Aib
  SITE 6: note = MISC_FEATURE - Xaa at position 6 is alpha-methyl-Phe
  SITE 13: note = MISC_FEATURE - Xaa at position 13 is alpha-methyl-Leu
  MOD_RES 17: note = Lys at position 17 is chemically modified by conjugation of the epsilon-amino group of the Lys side chain with (2-[2-(2-amino-ethoxy)-ethoxy]-acetyl)2-(gamma-Glu)-CO-(CH2)18-CO 2H
  SITE 20: note = MISC_FEATURE - Xaa at position 20 is Aib
  MOD_RES 39: note = Ser at position 39 is amidated
YXEGTXTSDYSIXLDEKAQXAFIEYLIEGGPSSGAPPPS

SEQ ID NO: 63 - protein, 39 aa, synthetic construct
  REGION 1..39: note = Synthetic Construct
  SITE 2: note = MISC_FEATURE - Xaa at position 2 is Aib
  SITE 6: note = MISC_FEATURE - Xaa at position 6 is alpha-methyl-Phe(2F)
  SITE 13: note = MISC_FEATURE - Xaa at position 13 is alpha-methyl-Leu
  MOD_RES 17: note = Lys at position 17 is chemically modified by conjugation of the epsilon-amino group of the Lys side chain with (2-[2-(2-amino-ethoxy)-ethoxy]-acetyl)2-(gamma-Glu)-CO-(CH2)18-CO 2H
  SITE 20: note = MISC_FEATURE - Xaa at position 20 is Aib
  MOD_RES 39: note = Ser at position 39 is amidated
YXEGTXTSDYSIXLDEKAQXEFIEYLIEGGPSSGAPPPS

SEQ ID NO: 64 - protein, 39 aa, synthetic construct
  REGION 1..39: note = Synthetic Construct
  SITE 2: note = MISC_FEATURE - Xaa at position 2 is Aib
  SITE 3: note = MISC_FEATURE - Xaa at position 3 is cTA
  SITE 6: note = MISC_FEATURE - Xaa at position 6 is alpha-methyl-Phe
  SITE 13: note = MISC_FEATURE - Xaa at position 13 is alpha-methyl-Leu
  MOD_RES 17: note = Lys at position 17 is chemically modified by conjugation of the epsilon-amino group of the Lys side chain with (2-[2-(2-amino-ethoxy)-ethoxy]-acetyl)2-(gamma-Glu)-CO-(CH2)18-CO 2H
  SITE 20: note = MISC_FEATURE - Xaa at position 20 is Aib
  MOD_RES 39: note = Ser at position 39 is amidated
YXXGTXTSDYSIXLDEKAQXAFIEYLIEGGPSSGAPPPS

SEQ ID NO: 65 - protein, 34 aa, synthetic construct
  REGION 1..34: note = Synthetic Construct
  SITE 2: note = MISC_FEATURE - Xaa at position 2 is Aib
  SITE 6: note = MISC_FEATURE - Xaa at position 6 is alpha-methyl-Phe
  SITE 13: note = MISC_FEATURE - Xaa at position 13 is alpha-methyl-Leu
  MOD_RES 17: note = Lys at position 17 is chemically modified by conjugation of the epsilon-amino group of the Lys side chain with (2-[2-(2-amino-ethoxy)-ethoxy]-acetyl)2-(gamma-Glu)-CO-(CH2)18-CO 2H
  SITE 20: note = MISC_FEATURE - Xaa at position 20 is Aib
  MOD_RES 34: note = Gly at position 34 is amidated
YXEGTXTSDYSIXLDKKAQXEFIEYLIEGGPSSG

SEQ ID NO: 66 - protein, 39 aa, synthetic construct; identical to SEQ ID NO: 41
  REGION 1..39: note = Synthetic Construct
  SITE 2: note = MISC_FEATURE - Xaa at position 2 is Aib
  SITE 6: note = MISC_FEATURE - Xaa at position 6 is alpha-methyl-Phe
  SITE 13: note = MISC_FEATURE - Xaa at position 13 is alpha-methyl-Leu
  MOD_RES 17: note = Lys at position 17 is chemically modified by conjugation of the epsilon-amino group of the Lys side chain with (2-[2-(2-amino-ethoxy)-ethoxy]-acetyl)2-(gamma-Glu)2-CO-(CH2)18-C O2H
  SITE 20: note = MISC_FEATURE - Xaa at position 20 is Aib
  MOD_RES 39: note = Ser at position 39 is amidated

SEQ ID NO: 67 - protein, 39 aa, synthetic construct
  REGION 1..39: note = Synthetic Construct
  SITE 2: note = MISC_FEATURE - Xaa at position 2 is Aib
  SITE 6: note = MISC_FEATURE - Xaa at position 6 is alpha-methyl-Phe
  SITE 13: note = MISC_FEATURE - Xaa at position 13 is alpha-methyl-Leu
  MOD_RES 17: note = Lys at position 17 is chemically modified by conjugation of the epsilon-amino group of the Lys side chain with (2-[2-(2-amino-ethoxy)-ethoxy]-acetyl)2-(gamma-Glu)-CO-(CH2)18-CO 2H
  SITE 20: note = MISC_FEATURE - Xaa at position 20 is Aib
  MOD_RES 39: note = Ser at position 39 is amidated
YXEGTXTSDYSIXLDKKAQXAFIEYLIEAGPSSGAPPPS

SEQ ID NO: 68 - protein, 39 aa, synthetic construct
  REGION 1..39: note = Synthetic Construct
  SITE 2: note = MISC_FEATURE - Xaa at position 2 is Aib
  SITE 6: note = MISC_FEATURE - Xaa at position 6 is alpha-methyl-Phe
  MOD_RES 17: note = Lys at position 17 is chemically modified by conjugation of the epsilon-amino group of the Lys side chain with (2-[2-(2-amino-ethoxy)-ethoxy]-acetyl)2-(gamma-Glu)-CO-(CH2)18-CO 2H
  SITE 20: note = MISC_FEATURE - Xaa at position 20 is Aib
  MOD_RES 39: note = Ser at position 39 is amidated
YXEGTXTSDHSILLDKKAQXAFIEYLIEGGPSSGAPPPS

SEQ ID NO: 69 - protein, 39 aa, synthetic construct
  REGION 1..39: note = Synthetic Construct
  SITE 2: note = MISC_FEATURE - Xaa at position 2 is Aib
  SITE 6: note = MISC_FEATURE - Xaa at position 6 is alpha-methyl-Phe
  MOD_RES 17: note = Lys at position 17 is chemically modified by conjugation of the epsilon-amino group of the Lys side chain with (2-[2-(2-amino-ethoxy)-ethoxy]-acetyl)2-(gamma-Glu)-CO-(CH2)18-CO 2H
  SITE 20: note = MISC_FEATURE - Xaa at position 20 is Aib
  MOD_RES 39: note = Ser at position 39 is amidated
YXEGTXTSDLSILLDKKAQXAFIEYLIEGGPSSGAPPPS

SEQ ID NO: 70 - protein, 39 aa, synthetic construct
  REGION 1..39: note = Synthetic Construct
  SITE 2: note = MISC_FEATURE - Xaa at position 2 is Aib
  SITE 6: note = MISC_FEATURE - Xaa at position 6 is alpha-methyl-Phe
  SITE 13: note = MISC_FEATURE - Xaa at position 13 is alpha-methyl-Leu
  MOD_RES 17: note = Lys at position 17 is chemically modified by conjugation of the epsilon-amino group of the Lys side chain with (2-[2-(2-amino-ethoxy)-ethoxy]-acetyl)2-(gamma-Glu)-CO-(CH2)18-CO 2H
  SITE 20: note = MISC_FEATURE - Xaa at position 20 is Aib
  SITE 21: note = MISC_FEATURE - Xaa at position 21 is Aad
  MOD_RES 39: note = Ser at position 39 is amidated
YXEGTXTSDYSIXLDKKAQXXFIEYLIEGGPSSGAPPPS

SEQ ID NO: 71 - protein, 39 aa, synthetic construct
  REGION 1..39: note = Synthetic Construct
  SITE 2: note = MISC_FEATURE - Xaa at position 2 is Aib
  SITE 6: note = MISC_FEATURE - Xaa at position 6 is alpha-methyl-Phe
  SITE 13: note = MISC_FEATURE - Xaa at position 13 is alpha-methyl-Leu
  MOD_RES 17: note = Lys at position 17 is chemically modified by conjugation of the epsilon-amino group of the Lys side chain with (2-[2-(2-amino-ethoxy)-ethoxy]-acetyl)2-(gamma-Glu)-CO-(CH2)18-CO 2H
  SITE 20: note = MISC_FEATURE - Xaa at position 20 is Aib
  MOD_RES 39: note = Ser at position 39 is amidated
YXEGTXTSDYSIXLDKKAQXTFIEYLIEGGPSSGAPPPS

SEQ ID NO: 72 - protein, 39 aa, synthetic construct
  REGION 1..39: note = Synthetic Construct
  SITE 2: note = MISC_FEATURE - Xaa at position 2 is Aib
  SITE 6: note = MISC_FEATURE - Xaa at position 6 is alpha-methyl-Phe
  SITE 13: note = MISC_FEATURE - Xaa at position 13 is alpha-methyl-Leu
  MOD_RES 17: note = Lys at position 17 is chemically modified by conjugation of the epsilon-amino group of the Lys side chain with (2-[2-(2-amino-ethoxy)-ethoxy]-acetyl)2-(gamma-Glu)-CO-(CH2)18-CO 2H
  SITE 20: note = MISC_FEATURE - Xaa at position 20 is Aib
  MOD_RES 39: note = Ser at position 39 is amidated
YXEGTXTSDYSIXLDKKAQXDFIEYLIEGGPSSGAPPPS

SEQ ID NO: 73 - protein, 39 aa, synthetic construct; identical to SEQ ID NO: 70
  REGION 1..39: note = Synthetic Construct
  SITE 2: note = MISC_FEATURE - Xaa at position 2 is Aib
  SITE 6: note = MISC_FEATURE - Xaa at position 6 is alpha-methyl-Phe
  SITE 13: note = MISC_FEATURE - Xaa at position 13 is alpha-methyl-Leu
  MOD_RES 17: note = Lys at position 17 is chemically modified by conjugation of the epsilon-amino group of the Lys side chain with (2-[2-(2-amino-ethoxy)-ethoxy]-acetyl)2-(gamma-Glu)-CO-(CH2)18-CO 2H
  SITE 20: note = MISC_FEATURE - Xaa at position 20 is Aib
  SITE 21: note = MISC_FEATURE - Xaa at position 21 is Aib
  MOD_RES 39: note = Ser at position 39 is amidated

SEQ ID NO: 74 - protein, 39 aa, synthetic construct
  REGION 1..39: note = Synthetic Construct
  SITE 2: note = MISC_FEATURE - Xaa at position 2 is Aib
  SITE 6: note = MISC_FEATURE - Xaa at position 6 is alpha-methyl-Phe
  SITE 13: note = MISC_FEATURE - Xaa at position 13 is alpha-methyl-Leu
  MOD_RES 17: note = Lys at position 17 is chemically modified by conjugation of the epsilon-amino group of the Lys side chain with (2-[2-(2-amino-ethoxy)-ethoxy]-acetyl)2-(gamma-Glu)-CO-(CH2)18-CO 2H
  SITE 21: note = MISC_FEATURE - Xaa at position 21 is Aib
  MOD_RES 39: note = Ser at position 39 is amidated
YXEGTXTSDYSIXLDKKAQHXFIEYLIEGGPSSGAPPPS

SEQ ID NO: 75 - protein, 39 aa, synthetic construct; identical to SEQ ID NO: 10
  REGION 1..39: note = Synthetic Construct
  SITE 2: note = MISC_FEATURE - Xaa at position 2 is Aib
  SITE 6: note = MISC_FEATURE - Xaa at position 6 is alpha-methyl-Phe(2F)
  SITE 13: note = MISC_FEATURE - Xaa at position 13 is alpha-methyl-Leu
  MOD_RES 17: note = Lys at position 17 is chemically modified by conjugation of the epsilon-amino group of the Lys side chain with (2-[2-(2-amino-ethoxy)-ethoxy]-acetyl)2-(gamma-Glu)-CO-(CH2)18-CO 2H
  SITE 20: note = MISC_FEATURE - Xaa at position 20 is Aib
  SITE 24: note = MISC_FEATURE - Xaa at position 24 is Aad
  MOD_RES 39: note = Ser at position 39 is amidated

SEQ ID NO: 76 - protein, 39 aa, synthetic construct
  REGION 1..39: note = Synthetic Construct
  SITE 2: note = MISC_FEATURE - Xaa at position 2 is Aib
  SITE 6: note = MISC_FEATURE - Xaa at position 6 is alpha-methyl-Phe(2F)
  SITE 13: note = MISC_FEATURE - Xaa at position 13 is alpha-methyl-Leu
  MOD_RES 17: note = Lys at position 17 is chemically modified by conjugation of the epsilon-amino group of the Lys side chain with (2-[2-(2-amino-ethoxy)-ethoxy]-acetyl)2-(gamma-Glu)-CO-(CH2)18-CO 2H
  SITE 20: note = MISC_FEATURE - Xaa at position 20 is Aib
  MOD_RES 39: note = Ser at position 39 is amidated
YXEGTXTSDYSIXLDEKAQXEFIAYLIEGGPSSGAPPPS

SEQ ID NO: 77 - protein, 39 aa, synthetic construct
  REGION 1..39: note = Synthetic Construct
  SITE 2: note = MISC_FEATURE - Xaa at position 2 is Aib
  SITE 6: note = MISC_FEATURE - Xaa at position 6 is alpha-methyl-Phe(2F)
  SITE 13: note = MISC_FEATURE - Xaa at position 13 is alpha-methyl-Leu
  MOD_RES 17: note = Lys at position 17 is chemically modified by conjugation of the epsilon-amino group of the Lys side chain with (2-[2-(2-amino-ethoxy)-ethoxy]-acetyl)2-(gamma-Glu)-CO-(CH2)18-CO 2H
  SITE 20: note = MISC_FEATURE - Xaa at position 20 is Aib
  MOD_RES 39: note = Ser at position 39 is amidated
YXEGTXTSDYSIXLDEKAQXEFIVYLIEGGPSSGAPPPS

SEQ ID NO: 78 - protein, 39 aa, synthetic construct
  REGION 1..39: note = Synthetic Construct
  SITE 2: note = MISC_FEATURE - Xaa at position 2 is Aib
  SITE 6: note = MISC_FEATURE - Xaa at position 6 is alpha-methyl-Phe(2F)
  SITE 13: note = MISC_FEATURE - Xaa at position 13 is alpha-methyl-Leu
  MOD_RES 17: note = Lys at position 17 is chemically modified by conjugation of the epsilon-amino group of the Lys side chain with (2-[2-(2-amino-ethoxy)-ethoxy]-acetyl)2-(gamma-Glu)-CO-(CH2)18-CO 2H
  SITE 20: note = MISC_FEATURE - Xaa at position 20 is Aib
  MOD_RES 39: note = Ser at position 39 is amidated
YXEGTXTSDYSIXLDEKAQXEFISYLIEGGPSSGAPPPS

SEQ ID NO: 79 - protein, 39 aa, synthetic construct
  REGION 1..39: note = Synthetic Construct
  SITE 2: note = MISC_FEATURE - Xaa at position 2 is Aib
  SITE 6: note = MISC_FEATURE - Xaa at position 6 is alpha-methyl-Phe(2F)
  SITE 13: note = MISC_FEATURE - Xaa at position 13 is alpha-methyl-Leu
  MOD_RES 17: note = Lys at position 17 is chemically modified by conjugation of the epsilon-amino group of the Lys side chain with (2-[2-(2-amino-ethoxy)-ethoxy]-acetyl)2-(gamma-Glu)-CO-(CH2)18-CO 2H
  SITE 20: note = MISC_FEATURE - Xaa at position 20 is Aib
  MOD_RES 39: note = Ser at position 39 is amidated
YXEGTXTSDYSIXLDEKAQXEFIPYLIEGGPSSGAPPPS

SEQ ID NO: 80 - protein, 39 aa, synthetic construct; identical to SEQ ID NO: 10
  REGION 1..39: note = Synthetic Construct
  SITE 2: note = MISC_FEATURE - Xaa at position 2 is Aib
  SITE 6: note = MISC_FEATURE - Xaa at position 6 is alpha-methyl-Phe(2F)
  SITE 13: note = MISC_FEATURE - Xaa at position 13 is alpha-methyl-Leu
  MOD_RES 17: note = Lys at position 17 is chemically modified by conjugation of the epsilon-amino group of the Lys side chain with (2-[2-(2-amino-ethoxy)-ethoxy]-acetyl)2-(gamma-Glu)-CO-(CH2)18-CO 2H
  SITE 20: note = MISC_FEATURE - Xaa at position 20 is Aib
  SITE 24: note = MISC_FEATURE - Xaa at position 24 is Aib
  MOD_RES 39: note = Ser at position 39 is amidated

SEQ ID NO: 81 - protein, 39 aa, synthetic construct
  REGION 1..39: note = Synthetic Construct
  SITE 2: note = MISC_FEATURE - Xaa at position 2 is Aib
  SITE 6: note = MISC_FEATURE - Xaa at position 6 is alpha-methyl-Phe(2F)
  SITE 13: note = MISC_FEATURE - Xaa at position 13 is alpha-methyl-Leu
  MOD_RES 17: note = Lys at position 17 is chemically modified by conjugation of the epsilon-amino group of the Lys side chain with (2-[2-(2-amino-ethoxy)-ethoxy]-acetyl)2-(gamma-Glu)-CO-(CH2)18-CO 2H
  SITE 20: note = MISC_FEATURE - Xaa at position 20 is Aib
  MOD_RES 39: note = Ser at position 39 is amidated
YXEGTXTSDYSIXLDEKAQXEFIHYLIEGGPSSGAPPPS

SEQ ID NO: 82 - protein, 39 aa, synthetic construct
  REGION 1..39: note = Synthetic Construct
  SITE 2: note = MISC_FEATURE - Xaa at position 2 is Aib
  SITE 6: note = MISC_FEATURE - Xaa at position 6 is alpha-methyl-Phe(2F)
  SITE 13: note = MISC_FEATURE - Xaa at position 13 is alpha-methyl-Leu
  MOD_RES 17: note = Lys at position 17 is chemically modified by conjugation of the epsilon-amino group of the Lys side chain with (2-[2-(2-amino-ethoxy)-ethoxy]-acetyl)2-(gamma-Glu)-CO-(CH2)18-CO 2H
  SITE 20: note = MISC_FEATURE - Xaa at position 20 is Aib
  MOD_RES 39: note = Ser at position 39 is amidated
YXEGTXTSDHSIXLDEKAQXEFIEYLIEGGPSSGAPPPS

SEQ ID NO: 83 - protein, 39 aa, synthetic construct
  REGION 1..39: note = Synthetic Construct
  SITE 2: note = MISC_FEATURE - Xaa at position 2 is Aib
  SITE 6: note = MISC_FEATURE - Xaa at position 6 is alpha-methyl-Phe(2F)
  SITE 10: note = MISC_FEATURE - Xaa at position 10 is cTA
  SITE 13: note = MISC_FEATURE - Xaa at position 13 is alpha-methyl-Leu
  MOD_RES 17: note = Lys at position 17 is chemically modified by conjugation of the epsilon-amino group of the Lys side chain with (2-[2-(2-amino-ethoxy)-ethoxy]-acetyl)2-(gamma-Glu)-CO-(CH2)18-CO 2H
  SITE 20: note = MISC_FEATURE - Xaa at position 20 is Aib
  MOD_RES 39: note = Ser at position 39 is amidated
YXEGTXTSDXSIXLDEKAQXEFIEYLIEGGPSSGAPPPS

SEQ ID NO: 84 - protein, 39 aa, synthetic construct; identical to SEQ ID NO: 83
  REGION 1..39: note = Synthetic Construct
  SITE 2: note = MISC_FEATURE - Xaa at position 2 is Aib
  SITE 6: note = MISC_FEATURE - Xaa at position 6 is alpha-methyl-Phe(2F)
  SITE 10: note = MISC_FEATURE - Xaa at position 10 is 3Pal
  SITE 13: note = MISC_FEATURE - Xaa at position 13 is alpha-methyl-Leu
  MOD_RES 17: note = Lys at position 17 is chemically modified by conjugation of the epsilon-amino group of the Lys side chain with (2-[2-(2-amino-ethoxy)-ethoxy]-acetyl)2-(gamma-Glu)-CO-(CH2)18-CO 2H
  SITE 20: note = MISC_FEATURE - Xaa at position 20 is Aib
  MOD_RES 39: note = Ser at position 39 is amidated

SEQ ID NO: 85 - protein, 34 aa, synthetic construct
  REGION 1..34: note = Synthetic Construct
  SITE 2: note = MISC_FEATURE - Xaa at position 2 is Aib
  SITE 6: note = MISC_FEATURE - Xaa at position 6 is alpha-methyl-Phe(2F)
  SITE 13: note = MISC_FEATURE - Xaa at position 13 is alpha-methyl-Leu
  MOD_RES 17: note = Lys at position 17 is chemically modified by conjugation of the epsilon-amino group of the Lys side chain with (2-[2-(2-amino-ethoxy)-ethoxy]-acetyl)2-(gamma-Glu)-CO-(CH2)18-CO 2H
  SITE 20: note = MISC_FEATURE - Xaa at position 20 is Aib
  SITE 24: note = MISC_FEATURE - Xaa at position 24 is D-Glu
  MOD_RES 34: note = Gly at position 34 is amidated
YXEGTXTSDHSIXLDEKAQXTFIXYLIEGGPSSG

SEQ ID NO: 86 - protein, 39 aa, synthetic construct
  REGION 1..39: note = Synthetic Construct
  SITE 2: note = MISC_FEATURE - Xaa at position 2 is Aib
  SITE 6: note = MISC_FEATURE - Xaa at position 6 is alpha-methyl-Phe(2F)
  SITE 13: note = MISC_FEATURE - Xaa at position 13 is alpha-methyl-Leu
  MOD_RES 17: note = Lys at position 17 is chemically modified by conjugation of the epsilon-amino group of the Lys side chain with (2-[2-(2-amino-ethoxy)-ethoxy]-acetyl)2-(gamma-Glu)-CO-(CH2)18-CO 2H
  SITE 20: note = MISC_FEATURE - Xaa at position 20 is Aib
  SITE 24: note = MISC_FEATURE - Xaa at position 24 is D-Glu
  MOD_RES 39: note = Ser at position 39 is amidated
YXEGTXTSDHSIXLDEKAQXTFIXYLIEGGPSSGAPPPS

SEQ ID NO: 87 - protein, 39 aa, synthetic construct; identical to SEQ ID NO: 86
  REGION 1..39: note = Synthetic Construct
  SITE 2: note = MISC_FEATURE - Xaa at position 2 is Aib
  SITE 6: note = MISC_FEATURE - Xaa at position 6 is alpha-methyl-Phe(2F)
  SITE 13: note = MISC_FEATURE - Xaa at position 13 is alpha-methyl-Leu
  MOD_RES 17: note = Lys at position 17 is chemically modified by conjugation of the epsilon-amino group of the Lys side chain with (2-[2-(2-amino-ethoxy)-ethoxy]-acetyl)2-(gamma-Glu)-CO-(CH2)16-CO 2H
  SITE 20: note = MISC_FEATURE - Xaa at position 20 is Aib
  SITE 24: note = MISC_FEATURE - Xaa at position 24 is D-Glu
  MOD_RES 39: note = Ser at position 39 is amidated

SEQ ID NO: 88 - protein, 39 aa, synthetic construct
  REGION 1..39: note = Synthetic Construct
  SITE 2: note = MISC_FEATURE - Xaa at position 2 is Aib
  SITE 6: note = MISC_FEATURE - Xaa at position 6 is alpha-methyl-Phe(2F)
  SITE 13: note = MISC_FEATURE - Xaa at position 13 is alpha-methyl-Leu
  SITE 16: note = MISC_FEATURE - Xaa at position 16 is Orn
  MOD_RES 17: note = Lys at position 17 is chemically modified by conjugation of the epsilon-amino group of the Lys side chain with (2-[2-(2-amino-ethoxy)-ethoxy]-acetyl)2-(gamma-Glu)-CO-(CH2)18-CO 2H
  SITE 20: note = MISC_FEATURE - Xaa at position 20 is Aib
  SITE 24: note = MISC_FEATURE - Xaa at position 24 is D-Glu
  MOD_RES 39: note = Ser at position 39 is amidated
YXEGTXTSDHSIXLDXKAQXTFIXYLIEGGPSSGAPPPS

SEQ ID NO: 89 - protein, 39 aa, synthetic construct; identical to SEQ ID NO: 88
  REGION 1..39: note = Synthetic Construct
  SITE 2: note = MISC_FEATURE - Xaa at position 2 is Aib
  SITE 6: note = MISC_FEATURE - Xaa at position 6 is alpha-methyl-Phe(2F)
  SITE 13: note = MISC_FEATURE - Xaa at position 13 is alpha-methyl-Leu
  SITE 16: note = MISC_FEATURE - Xaa at position 16 is Dab
  MOD_RES 17: note = Lys at position 17 is chemically modified by conjugation of the epsilon-amino group of the Lys side chain with (2-[2-(2-amino-ethoxy)-ethoxy]-acetyl)2-(gamma-Glu)-CO-(CH2)18-CO 2H
  SITE 20: note = MISC_FEATURE - Xaa at position 20 is a Aib
  SITE 24: note = MISC_FEATURE - Xaa at position 24 is D-Glu
  MOD_RES 39: note = Ser at position 39 is amidated

SEQ ID NO: 90 - protein, 39 aa, synthetic construct; identical to SEQ ID NO: 88
  REGION 1..39: note = Synthetic Construct
  SITE 2: note = MISC_FEATURE - Xaa at position 2 is Aib
  SITE 6: note = MISC_FEATURE - Xaa at position 6 is alpha-methyl-Phe(2F)
  SITE 13: note = MISC_FEATURE - Xaa at position 13 is alpha-methyl-Leu
  SITE 16: note = MISC_FEATURE - Xaa at position 16 is Dap
  MOD_RES 17: note = Lys at position 17 is chemically modified by conjugation of the epsilon-amino group of the Lys side chain with (2-[2-(2-amino-ethoxy)-ethoxy]-acetyl)2-(gamma-Glu)-CO-(CH2)18-CO 2H
  SITE 20: note = MISC_FEATURE - Xaa at position 20 is Aib
  SITE 24: note = MISC_FEATURE - Xaa at position 24 is D-Glu
  MOD_RES 39: note = Ser at position 39 is amidated

SEQ ID NO: 91 - protein, 39 aa, synthetic construct; identical to SEQ ID NO: 86
  REGION 1..39: note = Synthetic Construct
  SITE 2: note = MISC_FEATURE - Xaa at position 2 is Aib
  SITE 6: note = MISC_FEATURE - Xaa at position 6 is alpha-methyl-Phe(2F)
  SITE 13: note = MISC_FEATURE - Xaa at position 13 is alpha-methyl-Leu
  MOD_RES 17: note = Lys at position 17 is chemically modified by conjugation of the epsilon-amino group of the Lys side chain with (2-[2-(2-amino-ethoxy)-ethoxy]-acetyl)2-CO-(CH2)18-CO2H
  SITE 20: note = MISC_FEATURE - Xaa at position 20 is Aib
  SITE 24: note = MISC_FEATURE - Xaa at position 24 is D-Glu
  MOD_RES 39: note = Ser at position 39 is amidated

SEQ ID NO: 92 - protein, 39 aa, synthetic construct; identical to SEQ ID NO: 86
  REGION 1..39: note = Synthetic Construct
  SITE 2: note = MISC_FEATURE - Xaa at position 2 is Aib
  SITE 6: note = MISC_FEATURE - Xaa at position 6 is alpha-methyl-Phe(2F)
  SITE 13: note = MISC_FEATURE - Xaa at position 13 is alpha-methyl-Leu
  MOD_RES 17: note = Lys at position 17 is chemically modified by conjugation of the epsilon-amino group of the Lys side chain with (2-[2-(2-amino-ethoxy)-ethoxy]-acetyl)2-(epsilon-Lys)-CO-(CH2)16- CO2H
  SITE 20: note = MISC_FEATURE - Xaa at position 20 is Aib
  SITE 24: note = MISC_FEATURE - Xaa at position 24 is D-Glu
  MOD_RES 39: note = Ser at position 39 is amidated

SEQ ID NO: 93 - protein, 39 aa, synthetic construct
  REGION 1..39: note = Synthetic Construct
  SITE 2: note = MISC_FEATURE - Xaa at position 2 is Aib
  SITE 6: note = MISC_FEATURE - Xaa at position 6 is alpha-methyl-Phe(2F)
  SITE 13: note = MISC_FEATURE - Xaa at position 13 is alpha-methyl-Leu
  MOD_RES 17: note = Lys at position 17 is chemically modified by conjugation of the epsilon-amino group of the Lys side chain with (2-[2-(2-amino-ethoxy)-ethoxy]-acetyl)2-(gamma-Glu)-CO-(CH2)14-CO 2H
  SITE 20: note = MISC_FEATURE - Xaa at position 20 is Aib
  SITE 24: note = MISC_FEATURE - Xaa at position 24 is D-Glu
  MOD_RES 39: note = Ser at position 39 is amidated
YXEGTXTSDHSIXLDEKAQXHFIXYLIEGGPSSGAPPPS

SEQ ID NO: 94 - protein, 34 aa, synthetic construct
  REGION 1..34: note = Synthetic Construct
  SITE 2: note = MISC_FEATURE - Xaa at position 2 is Aib
  SITE 6: note = MISC_FEATURE - Xaa at position 6 is alpha-methyl-Phe(2F)
  SITE 13: note = MISC_FEATURE - Xaa at position 13 is alpha-methyl-Leu
  MOD_RES 17: note = Lys at position 17 is chemically modified by conjugation of the epsilon-amino group of the Lys side chain with (2-[2-(2-amino-ethoxy)-ethoxy]-acetyl)2-(gamma-Glu)-CO-(CH2)16-CO 2H
  SITE 20: note = MISC_FEATURE - Xaa at position 20 is Aib
  SITE 24: note = MISC_FEATURE - Xaa at position 24 is D-Glu
  MOD_RES 34: note = Gly at position 34 is amidated
YXEGTXTSDHSIXLDEKAQXHFIXYLIEGGPSSG

SEQ ID NO: 95 - protein, 30 aa, synthetic construct
  REGION 1..30: note = Synthetic Construct
  SITE 2: note = MISC_FEATURE - Xaa at position 2 is Aib
  SITE 6: note = MISC_FEATURE - Xaa at position 6 is alpha-methyl-Phe(2F)
  SITE 13: note = MISC_FEATURE - Xaa at position 13 is alpha-methyl-Leu
  MOD_RES 17: note = Lys at position 17 is chemically modified by conjugation of the epsilon-amino group of the Lys side chain with (2-[2-(2-amino-ethoxy)-ethoxy]-acetyl)2-(gamma-Glu)-CO-(CH2)16-CO 2H
  SITE 20: note = MISC_FEATURE - Xaa at position 20 is Aib
  SITE 24: note = MISC_FEATURE - Xaa at position 24 is D-Glu
  MOD_RES 30: note = Gly at position 30 is amidated
YXEGTXTSDHSIXLDEKAQXHFIXYLIEGG

SEQ ID NO: 96 - protein, 39 aa, synthetic construct
  REGION 1..39: note = Synthetic Construct
  SITE 2: note = MISC_FEATURE - Xaa at position 2 is Aib
  SITE 6: note = MISC_FEATURE - Xaa at position 6 is alpha-methyl-Phe(2F)
  SITE 10: note = MISC_FEATURE - Xaa at position 10 is 3Pal
  SITE 13: note = MISC_FEATURE - Xaa at position 13 is alpha-methyl-Leu
  MOD_RES 17: note = Lys at position 17 is chemically modified by conjugation of the epsilon-amino group of the Lys side chain with (2-[2-(2-amino-ethoxy)-ethoxy]-acetyl)2-(gamma-Glu)-CO-(CH2)18-CO 2H
  SITE 20: note = MISC_FEATURE - Xaa at position 20 is Aib
  SITE 24: note = MISC_FEATURE - Xaa at position 24 is D-Glu
  MOD_RES 39: note = Ser at position 39 is amidated
YXEGTXTSDXSIXLDEKAQXEFIXYLIEGGPSSGAPPPS

SEQ ID NO: 97 - protein, 39 aa, synthetic construct; identical to SEQ ID NO: 96
  REGION 1..39: note = Synthetic Construct
  SITE 2: note = MISC_FEATURE - Xaa at position 2 is Aib
  SITE 6: note = MISC_FEATURE - Xaa at position 6 is alpha-methyl-Phe(2F)
  SITE 10: note = MISC_FEATURE - Xaa at position 10 is 4Pal
  SITE 13: note = MISC_FEATURE - Xaa at position 13 is alpha-methyl-Leu
  MOD_RES 17: note = Lys at position 17 is chemically modified by conjugation of the epsilon-amino group of the Lys side chain with (2-[2-(2-amino-ethoxy)-ethoxy]-acetyl)2-(gamma-Glu)-CO-(CH2)18-CO 2H
  SITE 20: note = MISC_FEATURE - Xaa at position 20 is Aib
  SITE 24: note = MISC_FEATURE - Xaa at position 24 is D-Glu
  MOD_RES 39: note = Ser at position 39 is amidated

SEQ ID NO: 98 - protein, 39 aa, synthetic construct
  REGION 1..39: note = Synthetic Construct
  SITE 2: note = MISC_FEATURE - Xaa at position 2 is Aib
  SITE 6: note = MISC_FEATURE - Xaa at position 6 is alpha-methyl-Phe(2F)
  SITE 13: note = MISC_FEATURE - Xaa at position 13 is alpha-methyl-Leu
  MOD_RES 17: note = Lys at position 17 is chemically modified by conjugation of the epsilon-amino group of the Lys side chain with (2-[2-(2-amino-ethoxy)-ethoxy]-acetyl)2-(gamma-Glu)-CO-(CH2)18-CO 2H
  SITE 20: note = MISC_FEATURE - Xaa at position 20 is Aib
  SITE 24: note = MISC_FEATURE - Xaa at position 24 is D-Glu
  MOD_RES 39: note = Ser at position 39 is amidated
YXEGTXTSDLSIXLDEKAQXEFIXYLIEGGPSSGAPPPS

SEQ ID NO: 99 - protein, 39 aa, synthetic construct
  REGION 1..39: note = Synthetic Construct
  SITE 2: note = MISC_FEATURE - Xaa at position 2 is Aib
  SITE 6: note = MISC_FEATURE - Xaa at position 6 is alpha-methyl-Phe(2F)
  SITE 13: note = MISC_FEATURE - Xaa at position 13 is alpha-methyl-Leu
  MOD_RES 17: note = Lys at position 17 is chemically modified by conjugation of the epsilon-amino group of the Lys side chain with (2-[2-(2-amino-ethoxy)-ethoxy]-acetyl)2-(gamma-Glu)-CO-(CH2)18-CO 2H
  SITE 20: note = MISC_FEATURE - Xaa at position 20 is Aib
  SITE 24: note = MISC_FEATURE - Xaa at position 24 is D-Glu
  MOD_RES 39: note = Ser at position 39 is amidated
YXEGTXTSDQSIXLDEKAQXEFIXYLIEGGPSSGAPPPS

SEQ ID NO: 100 - protein, 39 aa, synthetic construct; identical to SEQ ID NO: 96
  REGION 1..39: note = Synthetic Construct
  SITE 2: note = MISC_FEATURE - Xaa at position 2 is Aib
  SITE 6: note = MISC_FEATURE - Xaa at position 6 is alpha-methyl-Phe(2F)
  SITE 10: note = MISC_FEATURE - Xaa at position 10 is 4Pal
  SITE 13: note = MISC_FEATURE - Xaa at position 13 is alpha-methyl-Leu
  MOD_RES 17: note = Lys at position 17 is chemically modified by conjugation of the epsilon-amino group of the Lys side chain with (2-[2-(2-amino-ethoxy)-ethoxy]-acetyl)2-(gamma-Glu)-CO-(CH2)18-CO 2H
  SITE 20: note = MISC_FEATURE - Xaa at position 20 is Aib
  SITE 24: note = MISC_FEATURE - Xaa at position 24 is Aib
  MOD_RES 39: note = Ser at position 39 is amidated

SEQ ID NO: 101 - protein, 34 aa, synthetic construct
  REGION 1..34: note = Synthetic Construct
  SITE 2: note = MISC_FEATURE - Xaa at position 2 is alpha-methyl-Pro
  MOD_RES 17: note = Lys at position 17 is chemically modified by conjugation of the epsilon-amino group of the Lys side chain with (2-[2-(2-amino-ethoxy)-ethoxy]-acetyl)2-(gamma-Glu)-CO-(CH2)16-CO 2H
  MOD_RES 34: note = Gly at position 34 is amidated
YXEGTFTSDYSILLDEKAQQAFIEYLIEGGPSSG

SEQ ID NO: 102 - protein, 39 aa, synthetic construct
  REGION 1..39: note = Synthetic Construct
  SITE 2: note = MISC_FEATURE - Xaa at position 2 is Aib
  SITE 6: note = MISC_FEATURE - Xaa at position 6 is alpha-methyl-Phe(2F)
  SITE 10: note = MISC_FEATURE - Xaa at position 10 is 4Pal
  SITE 13: note = MISC_FEATURE - Xaa at position 13 is alpha-methyl-Leu
  MOD_RES 17: note = Lys at position 17 is chemically modified by conjugation of the epsilon-amino group of the Lys side chain with (2-[2-(2-Amino-ethoxy)-ethoxy]-acetyl)-(gamma-Glu)-(2-[2-(2-Amino -ethoxy)-ethoxy]-acetyl)-CO-(CH2)18-CO2H
  SITE 20: note = MISC_FEATURE - Xaa at position 20 is Aib
  SITE 24: note = MISC_FEATURE - Xaa at position 24 is D-Glu
  MOD_RES 39: note = Ser at position 39 is amidated
YXEGTXTSDXSIXLDKKAQXEFIXYLIEGGPSSGAPPPS

SEQ ID NO: 103 - protein, 39 aa, synthetic construct; identical to SEQ ID NO: 102
  REGION 1..39: note = Synthetic Construct
  SITE 2: note = MISC_FEATURE - Xaa at position 2 is Aib
  SITE 6: note = MISC_FEATURE - Xaa at position 6 is alpha-methyl-Phe(2F)
  SITE 10: note = MISC_FEATURE - Xaa at position 10 is 4Pal
  SITE 13: note = MISC_FEATURE - Xaa at position 13 is alpha-methyl-Leu
  MOD_RES 17: note = Lys at position 17 is chemically modified by conjugation of the epsilon-amino group of the Lys side chain with (2-[2-(2-amino-ethoxy)-ethoxy]-acetyl)2-(gamma-Glu)-CO-(CH2)18-CO 2H
  SITE 20: note = MISC_FEATURE - Xaa at position 20 is Aib
  SITE 24: note = MISC_FEATURE - Xaa at position 24 is D-Glu
  MOD_RES 39: note = Ser at position 39 is amidated

SEQ ID NO: 104 - protein, 39 aa, synthetic construct; identical to SEQ ID NO: 96
  REGION 1..39: note = Synthetic Construct
  SITE 2: note = MISC_FEATURE - Xaa at position 2 is Aib
  SITE 6: note = MISC_FEATURE - Xaa at position 6 is alpha-methyl-Phe(2F)
  SITE 10: note = MISC_FEATURE - Xaa at position 10 is 4Pal
  SITE 13: note = MISC_FEATURE - Xaa at position 13 is alpha-methyl-Leu
  MOD_RES 17: note = Lys at position 17 is chemically modified by conjugation of the epsilon-amino group of the Lys side chain with (2-[2-(2-amino-ethoxy)-ethoxy]-acetyl)2-(gamma-Glu)-CO-(CH2)16-CO 2H
  SITE 20: note = MISC_FEATURE - Xaa at position 20 is Aib
  SITE 24: note = MISC_FEATURE - Xaa at position 24 is D-Glu
  MOD_RES 39: note = Ser at position 39 is amidated

SEQ ID NO: 105 - protein, 39 aa, synthetic construct; identical to SEQ ID NO: 96
  REGION 1..39: note = Synthetic Construct
  SITE 2: note = MISC_FEATURE - Xaa at position 2 is Aib
  SITE 6: note = MISC_FEATURE - Xaa at position 6 is alpha-methyl-Phe(2F)
  SITE 10: note = MISC_FEATURE - Xaa at position 10 is 4Pal
  SITE 13: note = MISC_FEATURE - Xaa at position 13 is alpha-methyl-Leu
  MOD_RES 17: note = Lys at position 17 is chemically modified by conjugation of the epsilon-amino group of the Lys side chain with (2-[2-(2-amino-ethoxy)-ethoxy]-acetyl)2-CO-(CH2)16-CO2H
  SITE 20: note = MISC_FEATURE - Xaa at position 20 is Aib
  SITE 24: note = MISC_FEATURE - Xaa at position 24 is D-Glu
  MOD_RES 39: note = Ser at position 39 is amidated

SEQ ID NO: 106 - protein, 39 aa, synthetic construct; identical to SEQ ID NO: 96
  REGION 1..39: note = Synthetic Construct
  SITE 2: note = MISC_FEATURE - Xaa at position 2 is Aib
  SITE 6: note = MISC_FEATURE - Xaa at position 6 is alpha-methyl-Phe(2F)
  SITE 10: note = MISC_FEATURE - Xaa at position 10 is 4Pal
  SITE 13: note = MISC_FEATURE - Xaa at position 13 is alpha-methyl-Leu
  MOD_RES 17: note = Lys at position 17 is chemically modified by conjugation of the epsilon-amino group of the Lys side chain with (2-[2-(2-amino-ethoxy)-ethoxy]-acetyl)2-CO-(CH2)18-CO2H
  SITE 20: note = MISC_FEATURE - Xaa at position 20 is Aib
  SITE 24: note = MISC_FEATURE - Xaa at position 24 is D-Glu
  MOD_RES 39: note = Ser at position 39 is amidated

SEQ ID NO: 107 - protein, 39 aa, synthetic construct; identical to SEQ ID NO: 96
  REGION 1..39: note = Synthetic Construct
  SITE 2: note = MISC_FEATURE - Xaa at position 2 is Aib
  SITE 6: note = MISC_FEATURE - Xaa at position 6 is alpha-methyl-Phe(2F)
  SITE 10: note = MISC_FEATURE - Xaa at position 10 is 4Pal
  SITE 13: note = MISC_FEATURE - Xaa at position 13 is alpha-methyl-Leu
  MOD_RES 17: note = Lys at position 17 is chemically modified by conjugation of the epsilon-amino group of the Lys side chain with (2-[2-(2-Amino-ethoxy)-ethoxy]-acetyl)2-(epsilon-Lys)-CO-(CH2)18- CO2H
  SITE 20: note = MISC_FEATURE - Xaa at position 20 is Aib
  SITE 24: note = MISC_FEATURE - Xaa at position 24 is D-Glu
  MOD_RES 39: note = Ser at position 39 is amidated

SEQ ID NO: 108 - protein, 39 aa, synthetic construct; identical to SEQ ID NO: 10
  REGION 1..39: note = Synthetic Construct
  SITE 2: note = MISC_FEATURE - Xaa at position 2 is Aib
  SITE 6: note = MISC_FEATURE - Xaa at position 6 is alpha-methyl-Phe(2F)
  SITE 13: note = MISC_FEATURE - Xaa at position 13 is alpha-methyl-Leu
  MOD_RES 17: note = Lys at position 17 is chemically modified by conjugation of the epsilon-amino group of the Lys side chain with (2-[2-(2-amino-ethoxy)-ethoxy]-acetyl)2-(gamma-Glu)-CO-(CH2)14-CO 2H
  SITE 20: note = MISC_FEATURE - Xaa at position 20 is Aib
  SITE 24: note = MISC_FEATURE - Xaa at position 24 is D-Glu
  MOD_RES 39: note = Ser at position 39 is amidated

SEQ ID NO: 109 - protein, 39 aa, synthetic construct; identical to SEQ ID NO: 11
  REGION 1..39: note = Synthetic Construct
  SITE 2: note = MISC_FEATURE - Xaa at position 2 is Aib
  SITE 6: note = MISC_FEATURE - Xaa at position 6 is alpha-methyl-Phe(2F)
  SITE 13: note = MISC_FEATURE - Xaa at position 13 is alpha-methyl-Leu
  SITE 16: note = MISC_FEATURE - Xaa at position 16 is Dab
  MOD_RES 17: note = Lys at position 17 is chemically modified by conjugation of the epsilon-amino group of the Lys side chain with (2-[2-(2-amino-ethoxy)-ethoxy]-acetyl)2-(gamma-Glu)-CO-(CH2)16-CO 2H
  SITE 20: note = MISC_FEATURE - Xaa at position 20 is Aib
  SITE 24: note = MISC_FEATURE - Xaa at position 24 is D-Glu
  MOD_RES 39: note = Ser at position 39 is amidated

SEQ ID NO: 110 - protein, 39 aa, synthetic construct; identical to SEQ ID NO: 11
  REGION 1..39: note = Synthetic Construct
  SITE 2: note = MISC_FEATURE - Xaa at position 2 is Aib
  SITE 6: note = MISC_FEATURE - Xaa at position 6 is alpha-methyl-Phe(2F)
  SITE 13: note = MISC_FEATURE - Xaa at position 13 is alpha-methyl-Leu
  SITE 16: note = MISC_FEATURE - Xaa at position 16 is Dap
  MOD_RES 17: note = Lys at position 17 is chemically modified by conjugation of the epsilon-amino group of the Lys side chain with (2-[2-(2-amino-ethoxy)-ethoxy]-acetyl)2-(gamma-Glu)-CO-(CH2)16-CO 2H
  SITE 20: note = MISC_FEATURE - Xaa at position 20 is Aib
  SITE 24: note = MISC_FEATURE - Xaa at position 24 is D-Glu
  MOD_RES 39: note = Ser at position 39 is amidated

SEQ ID NO: 111 - protein, 39 aa, synthetic construct
  REGION 1..39: note = Synthetic Construct
  SITE 2: note = MISC_FEATURE - Xaa at position 2 is Aib
  SITE 6: note = MISC_FEATURE - Xaa at position 6 is alpha-methyl-Phe(2F)
  SITE 13: note = MISC_FEATURE - Xaa at position 13 is alpha-methyl-Leu
  MOD_RES 17: note = Lys at position 17 is chemically modified by conjugation of the epsilon-amino group of the Lys side chain with (2-[2-(2-Amino-ethoxy)-ethoxy]-acetyl)-(gamma-Glu)-(2-[2-(2-Amino -ethoxy)-ethoxy]-acetyl)-CO-(CH2)18-CO2H
  SITE 20: note = MISC_FEATURE - Xaa at position 20 is Aib
  SITE 24: note = MISC_FEATURE - Xaa at position 24 is D-Glu
  MOD_RES 39: note = Ser at position 39 is amidated
YXEGTXTSDYSIXLDKKAQXEFIXYLIEGGPSSGAPPPS

SEQ ID NO: 112 - protein, 39 aa, synthetic construct; identical to SEQ ID NO: 111
  REGION 1..39: note = Synthetic Construct
  SITE 2: note = MISC_FEATURE - Xaa at position 2 is Aib
  SITE 6: note = MISC_FEATURE - Xaa at position 6 is alpha-methyl-Phe(2F)
  SITE 13: note = MISC_FEATURE - Xaa at position 13 is alpha-methyl-Leu
  MOD_RES 17: note = Lys at position 17 is chemically modified by conjugation of the epsilon-amino group of the Lys side chain with (2-[2-(2-amino-ethoxy)-ethoxy]-acetyl)2-(gamma-Glu)-CO-(CH2)18-CO 2H
  SITE 20: note = MISC_FEATURE - Xaa at position 20 is Aib
  SITE 24: note = MISC_FEATURE - Xaa at position 24 is D-Glu
  MOD_RES 39: note = Ser at position 39 is amidated

SEQ ID NO: 113 - protein, 39 aa, synthetic construct; identical to SEQ ID NO: 10
  REGION 1..39: note = Synthetic Construct
  SITE 2: note = MISC_FEATURE - Xaa at position 2 is Aib
  SITE 6: note = MISC_FEATURE - Xaa at position 6 is alpha-methyl-Phe
  SITE 13: note = MISC_FEATURE - Xaa at position 13 is alpha-methyl-Leu
  MOD_RES 17: note = Lys at position 17 is chemically modified by conjugation of the epsilon-amino group of the Lys side chain with (2-[2-(2-amino-ethoxy)-ethoxy]-acetyl)2-(gamma-Glu)-CO-(CH2)16-CO 2H
  SITE 20: note = MISC_FEATURE - Xaa at position 20 is Aib
  SITE 24: note = MISC_FEATURE - Xaa at position 24 is D-Glu
  MOD_RES 39: note = Ser at position 39 is amidated

SEQ ID NO: 114 - protein, 39 aa, synthetic construct; identical to SEQ ID NO: 10
  REGION 1..39: note = Synthetic Construct
  SITE 2: note = MISC_FEATURE - Xaa at position 2 is Aib
  SITE 6: note = MISC_FEATURE - Xaa at position 6 is alpha-methyl-Phe(2F)
  SITE 13: note = MISC_FEATURE - Xaa at position 13 is alpha-methyl-Leu
  MOD_RES 17: note = Lys at position 17 is chemically modified by conjugation of the epsilon-amino group of the Lys side chain with (2-[2-(2-amino-ethoxy)-ethoxy]-acetyl)2-CO-(CH2)16-CO2H
  SITE 20: note = MISC_FEATURE - Xaa at position 20 is Aib
  SITE 24: note = MISC_FEATURE - Xaa at position 24 is D-Glu
  MOD_RES 39: note = Ser at position 39 is amidated

SEQ ID NO: 115 - protein, 39 aa, synthetic construct; identical to SEQ ID NO: 10
  REGION 1..39: note = Synthetic Construct
  SITE 2: note = MISC_FEATURE - Xaa at position 2 is Aib
  SITE 6: note = MISC_FEATURE - Xaa at position 6 is alpha-methyl-Phe(2F)
  SITE 13: note = MISC_FEATURE - Xaa at position 13 is alpha-methyl-Leu
  MOD_RES 17: note = Lys at position 17 is chemically modified by conjugation of the epsilon-amino group of the Lys side chain with (2-[2-(2-amino-ethoxy)-ethoxy]-acetyl)2-CO-(CH2)18-CO2H
  SITE 20: note = MISC_FEATURE - Xaa at position 20 is Aib
  SITE 24: note = MISC_FEATURE - Xaa at position 24 is D-Glu
  MOD_RES 39: note = Ser at position 39 is amidated

SEQ ID NO: 116 - protein, 39 aa, synthetic construct; identical to SEQ ID NO: 10
  REGION 1..39: note = Synthetic Construct
  SITE 2: note = MISC_FEATURE - Xaa at position 2 is Aib
  SITE 6: note = MISC_FEATURE - Xaa at position 6 is alpha-methyl-Phe(2F)
  SITE 13: note = MISC_FEATURE - Xaa at position 13 is alpha-methyl-Leu
  MOD_RES 17: note = Lys at position 17 is chemically modified by conjugation of the epsilon-amino group of the Lys side chain with (2-[2-(2-amino-ethoxy)-ethoxy]-acetyl)2-(epsilon-Lys)-CO-(CH2)18- CO2H
  SITE 20: note = MISC_FEATURE - Xaa at position 20 is Aib
  SITE 24: note = MISC_FEATURE - Xaa at position 24 is D-Glu
  MOD_RES 39: note = Ser at position 39 is amidated

SEQ ID NO: 117 - protein, 39 aa, synthetic construct; identical to SEQ ID NO: 11
  REGION 1..39: note = Synthetic Construct
  SITE 2: note = MISC_FEATURE - Xaa at position 2 is Aib
  SITE 6: note = MISC_FEATURE - Xaa at position 6 is alpha-methyl-Phe(2F)
  SITE 13: note = MISC_FEATURE - Xaa at position 13 is alpha-methyl-Leu
  SITE 16: note = MISC_FEATURE - Xaa at position 16 is Dab
  MOD_RES 17: note = Lys at position 17 is chemically modified by conjugation of the epsilon-amino group of the Lys side chain with (2-[2-(2-amino-ethoxy)-ethoxy]-acetyl)2-(gamma-Glu)-CO-(CH2)18-CO 2H
  SITE 20: note = MISC_FEATURE - Xaa at position 20 is Aib
  SITE 24: note = MISC_FEATURE - Xaa at position 24 is D-Glu
  MOD_RES 39: note = Ser at position 39 is amidated

SEQ ID NO: 118 - protein, 39 aa, synthetic construct; identical to SEQ ID NO: 11
  REGION 1..39: note = Synthetic Construct
  SITE 2: note = MISC_FEATURE - Xaa at position 2 is Aib
  SITE 6: note = MISC_FEATURE - Xaa at position 6 is alpha-methyl-Phe(2F)
  SITE 13: note = MISC_FEATURE - Xaa at position 13 is alpha-methyl-Leu
  SITE 16: note = MISC_FEATURE - Xaa at position 16 is Dap
  MOD_RES 17: note = Lys at position 17 is chemically modified by conjugation of the epsilon-amino group of the Lys side chain with (2-[2-(2-amino-ethoxy)-ethoxy]-acetyl)2-(gamma-Glu)-CO-(CH2)18-CO 2H
  SITE 20: note = MISC_FEATURE - Xaa at position 20 is Aib
  SITE 24: note = MISC_FEATURE - Xaa at position 24 is D-Glu
  MOD_RES 39: note = Ser at position 39 is amidated

SEQ ID NO: 119 - protein, 34 aa, synthetic construct
  REGION 1..34: note = Synthetic Construct
  SITE 2: note = MISC_FEATURE - Xaa at position 2 is Aib
  SITE 6: note = MISC_FEATURE - Xaa at position 6 is alpha-methyl-Phe(2F)
  SITE 13: note = MISC_FEATURE - Xaa at position 13 is alpha-methyl-Leu
  MOD_RES 17: note = Lys at position 17 is chemically modified by conjugation of the epsilon-amino group of the Lys side chain with (2-[2-(2-amino-ethoxy)-ethoxy]-acetyl)2-(gamma-Glu)-CO-(CH2)16-CO 2H
  SITE 20: note = MISC_FEATURE - Xaa at position 20 is Aib
  SITE 24: note = MISC_FEATURE - Xaa at position 24 is D-Glu
  MOD_RES 34: note = Gly at position 34 is amidated
YXEGTXTSDYSIXLDEKAQXEFIXYLIEGGPSSG

SEQ ID NO: 120 - protein, 30 aa, synthetic construct
  REGION 1..30: note = Synthetic Construct
  SITE 2: note = MISC_FEATURE - Xaa at position 2 is Aib
  SITE 6: note = MISC_FEATURE - Xaa at position 6 is alpha-methyl-Phe(2F)
  SITE 13: note = MISC_FEATURE - Xaa at position 13 is alpha-methyl-Leu
  MOD_RES 17: note = Lys at position 17 is chemically modified by conjugation of the epsilon-amino group of the Lys side chain with (2-[2-(2-amino-ethoxy)-ethoxy]-acetyl)2-(gamma-Glu)-CO-(CH2)16-CO 2H
  SITE 20: note = MISC_FEATURE - Xaa at position 20 is Aib
  SITE 24: note = MISC_FEATURE - Xaa at position 24 is D-Glu
  MOD_RES 30: note = Gly at position 30 is amidated
YXEGTXTSDYSIXLDEKAQXEFIXYLIEGG

SEQ ID NO: 121 - protein, 39 aa, synthetic construct; identical to SEQ ID NO: 10
  REGION 1..39: note = Synthetic Construct
  SITE 2: note = MISC_FEATURE - Xaa at position 2 is Aib
  SITE 6: note = MISC_FEATURE - Xaa at position 6 is alpha-methyl-Phe(2F)
  SITE 13: note = MISC_FEATURE - Xaa at position 13 is alpha-methyl-Leu
  MOD_RES 17: note = Lys at position 17 is chemically modified by conjugation of the epsilon-amino group of the Lys side chain with (2-[2-(2-amino-ethoxy)-ethoxy]-acetyl)2-(gamma-Glu)-CO-(CH2)16-CO 2H
  SITE 20: note = MISC_FEATURE - Xaa at position 20 is Aib
  SITE 24: note = MISC_FEATURE - Xaa at position 24 is D-Glu
  MOD_RES 39: note = Ser at position 39 is amidated

SEQ ID NO: 122 - protein, 39 aa, synthetic construct
  REGION 1..39: note = Synthetic Construct
  SITE 2: note = MISC_FEATURE - Xaa at position 2 is Aib
  SITE 6: note = MISC_FEATURE - Xaa at position 6 is alpha-methyl-Phe(2F)
  SITE 13: note = MISC_FEATURE - Xaa at position 13 is alpha-methyl-Leu
  MOD_RES 17: note = Lys at position 17 is chemically modified by conjugation of the epsilon-amino group of the Lys side chain with (2-[2-(2-amino-ethoxy)-ethoxy]-acetyl)2-(gamma-Glu)-CO-(CH2)18-CO 2H
  SITE 20: note = MISC_FEATURE - Xaa at position 20 is Aib
  SITE 24: note = MISC_FEATURE - Xaa at position 24 is D-Glu
  SITE 25: note = MISC_FEATURE - Xaa at position 25 alpha-methyl-Tyr
  MOD_RES 39: note = Ser at position 39 is amidated
YXEGTXTSDYSIXLDEKAQXEFIXXLIEGGPSSGAPPPS

SEQ ID NO: 123 - protein, 39 aa, synthetic construct
  REGION 1..39: note = Synthetic Construct
  SITE 2: note = MISC_FEATURE - Xaa at position 2 is Aib
  SITE 6: note = MISC_FEATURE - Xaa at position 6 is alpha-methyl-Phe(2F)
  SITE 13: note = MISC_FEATURE - Xaa at position 13 is alpha-methyl-Leu
  MOD_RES 17: note = Lys at position 17 is chemically modified by conjugation of the epsilon-amino group of the Lys side chain with (2-[2-(2-amino-ethoxy)-ethoxy]-acetyl)2-(gamma-Glu)-CO-(CH2)18-CO 2H
  SITE 20: note = MISC_FEATURE - Xaa at position 20 is Aib
  SITE 25: note = MISC_FEATURE - Xaa at position 25 is alpha-methyl-Tyr
  MOD_RES 39: note = Ser at position 39 is amidated
YXEGTXTSDYSIXLDEKAQXEFIEXLIEGGPSSGAPPPS

SEQ ID NO: 124 - protein, 39 aa, synthetic construct; identical to SEQ ID NO: 10
  REGION 1..39: note = Synthetic Construct
  SITE 2: note = MISC_FEATURE - Xaa at position 2 is Aib
  SITE 6: note = MISC_FEATURE - Xaa at position 6 is alpha-methyl-Phe(2F)
  SITE 13: note = MISC_FEATURE - Xaa at position 13 is Aib
  MOD_RES 17: note = Lys at position 17 is chemically modified by conjugation of the epsilon-amino group of the Lys side chain with (2-[2-(2-amino-ethoxy)-ethoxy]-acetyl)2-(gamma-Glu)-CO-(CH2)18-CO 2H
  SITE 20: note = MISC_FEATURE - Xaa at position 20 is Aib
  SITE 24: note = MISC_FEATURE - Xaa at position 24 is D-Glu
  MOD_RES 39: note = Ser at position 39 is amidated

SEQ ID NO: 125 - protein, 39 aa, synthetic construct; identical to SEQ ID NO: 10
  REGION 1..39: note = Synthetic Construct
  SITE 2: note = MISC_FEATURE - Xaa at position 2 is Aib
  SITE 6: note = MISC_FEATURE - Xaa at position 6 is alpha-methyl-Phe
  SITE 13: note = MISC_FEATURE - Xaa at position 13 is Aib
  MOD_RES 17: note = Lys at position 17 is chemically modified by conjugation of the epsilon-amino group of the Lys side chain with (2-[2-(2-amino-ethoxy)-ethoxy]-acetyl)2-(gamma-Glu)-CO-(CH2)18-CO 2H
  SITE 20: note = MISC_FEATURE - Xaa at position 20 is Aib
  SITE 24: note = MISC_FEATURE - Xaa at position 24 is D-Glu
  MOD_RES 39: note = Ser at position 39 is amidated

SEQ ID NO: 126 - protein, 39 aa, synthetic construct
  REGION 1..39: note = Synthetic Construct
  SITE 2: note = MISC_FEATURE - Xaa at position 2 is Aib
  SITE 6: note = MISC_FEATURE - Xaa at position 6 is alpha-methyl-Phe(2F)
  MOD_RES 17: note = Lys at position 17 is chemically modified by conjugation of the epsilon-amino group of the Lys side chain with (2-[2-(2-amino-ethoxy)-ethoxy]-acetyl)2-(gamma-Glu)-CO-(CH2)18-CO 2H
  SITE 20: note = MISC_FEATURE - Xaa at position 20 is Aib
  SITE 24: note = MISC_FEATURE - Xaa at position 24 is D-Glu
  MOD_RES 39: note = Ser at position 39 is amidated
YXEGTXTSDYSILLDEKAQXEFIXYLIEGGPSSGAPPPS

SEQ ID NO: 127 - protein, 39 aa, synthetic construct; identical to SEQ ID NO: 10
  REGION 1..39: note = Synthetic Construct
  SITE 2: note = MISC_FEATURE - Xaa at position 2 is Aib
  SITE 6: note = MISC_FEATURE - Xaa at position 6 is alpha-methyl-Phe
  SITE 13: note = MISC_FEATURE - Xaa at position 13 is alpha-methyl-Leu
  MOD_RES 17: note = Lys at position 17 is chemically modified by conjugation of the epsilon-amino group of the Lys side chain with (2-[2-(2-amino-ethoxy)-ethoxy]-acetyl)2-(gamma-Glu)-CO-(CH2)18-CO 2H
  SITE 20: note = MISC_FEATURE - Xaa at position 20 is Aib
  SITE 24: note = MISC_FEATURE - Xaa at position 24 is D-Glu
  MOD_RES 39: note = Ser at position 39 is amidated

SEQ ID NO: 128 - protein, 34 aa, synthetic construct
  REGION 1..34: note = Synthetic Construct
  SITE 2: note = MISC_FEATURE - Xaa at position 2 is Aib
  SITE 6: note = MISC_FEATURE - Xaa at position 6 is alpha-methyl-Phe
  SITE 13: note = MISC_FEATURE - Xaa at position 13 is alpha-methyl-Leu
  MOD_RES 17: note = Lys at position 17 is chemically modified by conjugation of the epsilon-amino group of the Lys side chain with (2-[2-(2-amino-ethoxy)-ethoxy]-acetyl)2-(gamma-Glu)-CO-(CH2)18-CO 2H
  SITE 20: note = MISC_FEATURE - Xaa at position 20 is Aib
  SITE 24: note = MISC_FEATURE - Xaa at position 24 is D-Glu
  MOD_RES 34: note = Gly at position 34 is amidated
YXEGTXTSDYSIXLDKKAQXEFIXYLIEGGPSSG

SEQ ID NO: 129 - protein, 39 aa, synthetic construct
  REGION 1..39: note = Synthetic Construct
  SITE 2: note = MISC_FEATURE - Xaa at position 2 is Aib
  SITE 6: note = MISC_FEATURE - Xaa at position 6 is alpha-methyl-Phe(2F)
  SITE 13: note = MISC_FEATURE - Xaa at position 13 is alpha-methyl-Leu
  MOD_RES 17: note = Lys at position 17 is chemically modified by conjugation of the epsilon-amino group of the Lys side chain with (2-[2-(2-amino-ethoxy)-ethoxy]-acetyl)2-(gamma-Glu)-CO-(CH2)18-CO 2H
  SITE 20: note = MISC_FEATURE - Xaa at position 20 is Aib
  SITE 24: note = MISC_FEATURE - Xaa at position 24 is D-Glu
  MOD_RES 39: note = Ser at position 39 is amidated
YXEGTXTSDYSIXLDHKAQXEFIXYLIEGGPSSGAPPPS

SEQ ID NO: 130 - protein, 39 aa, synthetic construct
  REGION 1..39: note = Synthetic Construct
  SITE 2: note = MISC_FEATURE - Xaa at position 2 is Aib
  SITE 6: note = MISC_FEATURE - Xaa at position 6 is alpha-methyl-Phe(2F)
  SITE 10: note = MISC_FEATURE - Xaa at position 10 is 4Pal
  SITE 13: note = MISC_FEATURE - Xaa at position 13 is alpha-methyl-Leu
  SITE 16: note = MISC_FEATURE - Xaa at position 16 is Dab
  MOD_RES 17: note = Lys at position 17 is chemically modified by conjugation of the epsilon-amino group of the Lys side chain with (2-[2-(2-amino-ethoxy)-ethoxy]-acetyl)2-(gamma-Glu)-CO-(CH2)16-CO 2H
  SITE 20: note = MISC_FEATURE - Xaa at position 20 is Aib
  SITE 24: note = MISC_FEATURE - Xaa at position 24 is D-Glu
  MOD_RES 39: note = Ser at position 39 is amidated
YXEGTXTSDXSIXLDXKAQXEFIXYLIEGGPSSGAPPPS

SEQ ID NO: 131 - protein, 39 aa, synthetic construct
  REGION 1..39: note = Synthetic Construct
  SITE 2: note = MISC_FEATURE - Xaa at position 2 is Aib
  SITE 6: note = MISC_FEATURE - Xaa at position 6 is alpha-methyl-Phe(2F)
  SITE 13: note = MISC_FEATURE - Xaa at position 13 is alpha-methyl-Leu
  SITE 16: note = MISC_FEATURE - Xaa at position 16 is Orn
  MOD_RES 17: note = Lys at position 17 is chemically modified by conjugation of the epsilon-amino group of the Lys side chain with (2-[2-(2-amino-ethoxy)-ethoxy]-acetyl)2-(gamma-Glu)-CO-(CH2)16-CO 2H
  SITE 20: note = MISC_FEATURE - Xaa at position 20 is Aib
  SITE 24: note = MISC_FEATURE - Xaa at position 24 is D-Glu
  SITE 25: note = MISC_FEATURE - Xaa at position 25 is alpha-methyl-Tyr
  MOD_RES 39: note = Ser at position 39 is amidated
YXEGTXTSDYSIXLDXKAQXEFIXXLIEGGPSSGAPPPS

SEQ ID NO: 132 - protein, 39 aa, synthetic construct
  REGION 1..39: note = Synthetic Construct
  SITE 2: note = MISC_FEATURE - Xaa at position 2 is Aib
  SITE 6: note = MISC_FEATURE - Xaa at position 6 is alpha-methyl-Phe(2F)
  SITE 13: note = MISC_FEATURE - Xaa at position 13 is alpha-methyl-Leu
  SITE 16: note = MISC_FEATURE - Xaa at position 16 is Orn
  MOD_RES 17: note = Lys at position 17 is chemically modified by conjugation of the epsilon-amino group of the Lys side chain with (2-[2-(2-amino-ethoxy)-ethoxy]-acetyl)2-(gamma-Glu)-CO-(CH2)16-CO 2H
  SITE 20: note = MISC_FEATURE - Xaa at position 20 is Aib
  SITE 24: note = MISC_FEATURE - Xaa at position 24 is D-Glu
  SITE 25: note = MISC_FEATURE - Xaa at position 25 is alpha-methyl-Tyr
  MOD_RES 39: note = Ser at position 39 is amidated
YXEGTXTSDLSIXLDXKAQXEFIXXLIEGGPSSGAPPPS

SEQ ID NO: 133 - protein, 39 aa, synthetic construct
  REGION 1..39: note = Synthetic Construct
  SITE 2: note = MISC_FEATURE - Xaa at position 2 is Aib
  SITE 6: note = MISC_FEATURE - Xaa at position 6 is alpha-methyl-Phe(2F)
  SITE 10: note = MISC_FEATURE - Xaa at position 10 is 4Pal
  SITE 13: note = MISC_FEATURE - Xaa at position 13 is alpha-methyl-Leu
  SITE 16: note = MISC_FEATURE - Xaa at position 16 is Orn
  MOD_RES 17: note = Lys at position 17 is chemically modified by conjugation of the epsilon-amino group of the Lys side chain with (2-[2-(2-amino-ethoxy)-ethoxy]-acetyl)2-(gamma-Glu)-CO-(CH2)16-CO 2H
  SITE 20: note = MISC_FEATURE - Xaa at position 20 is Aib
  SITE 24: note = MISC_FEATURE - Xaa at position 24 is D-Glu
  SITE 25: note = MISC_FEATURE - Xaa at position 25 is alpha-methyl-Tyr
  MOD_RES 39: note = Ser at position 39 is amidated
YXEGTXTSDXSIXLDXKAQXTFIXXLIEGGPSSGAPPPS

SEQ ID NO: 134 - protein, 39 aa, synthetic construct
  REGION 1..39: note = Synthetic Construct
  SITE 2: note = MISC_FEATURE - Xaa at position 2 is Aib
  SITE 6: note = MISC_FEATURE - Xaa at position 6 is alpha-methyl-Phe(2F)
  SITE 13: note = MISC_FEATURE - Xaa at position 13 is alpha-methyl-Leu
  SITE 16: note = MISC_FEATURE - Xaa at position 16 is Orn
  MOD_RES 17: note = Lys at position 17 is chemically modified by conjugation of the epsilon-amino group of the Lys side chain with (2-[2-(2-amino-ethoxy)-ethoxy]-acetyl)2-(gamma-Glu)-CO-(CH2)16-CO 2H
  SITE 20: note = MISC_FEATURE - Xaa at position 20 is Aib
  SITE 24: note = MISC_FEATURE - Xaa at position 24 is D-Glu
  SITE 25: note = MISC_FEATURE - Xaa at position 25 is alpha-methyl-Tyr
  MOD_RES 39: note = Ser at position 39 is amidated
YXEGTXTSDVSIXLDXKAQXTFIXXLIEGGPSSGAPPPS

SEQ ID NO: 135 - protein, 39 aa, synthetic construct
  REGION 1..39: note = Synthetic Construct
  SITE 2: note = MISC_FEATURE - Xaa at position 2 is Aib
  SITE 6: note = MISC_FEATURE - Xaa at position 6 is alpha-methyl-Phe(2F)
  SITE 13: note = MISC_FEATURE - Xaa at position 13 is alpha-methyl-Leu
  SITE 16: note = MISC_FEATURE - Xaa at position 16 is Orn
  MOD_RES 17: note = Lys at position 17 is chemically modified by conjugation of the epsilon-amino group of the Lys side chain with (2-[2-(2-amino-ethoxy)-ethoxy]-acetyl)2-(gamma-Glu)-CO-(CH2)16-CO 2H
  SITE 20: note = MISC_FEATURE - Xaa at position 20 is Aib
  SITE 24: note = MISC_FEATURE - Xaa at position 24 is D-Glu
  SITE 25: note = MISC_FEATURE - Xaa at position 25 is alpha-methyl-Tyr
  MOD_RES 39: note = Ser at position 39 is amidated
YXEGTXTSDVSIXLDXKAQXAFIXXLIEGGPSSGAPPPS

SEQ ID NO: 136 - protein, 39 aa, synthetic construct
  REGION 1..39: note = Synthetic Construct
  SITE 2: note = MISC_FEATURE - Xaa at position 2 is Aib
  SITE 6: note = MISC_FEATURE - Xaa at position 6 is alpha-methyl-Phe(2F)
  SITE 13: note = MISC_FEATURE - Xaa at position 13 is alpha-methyl-Leu
  SITE 16: note = MISC_FEATURE - Xaa at position 16 is Orn
  MOD_RES 17: note = Lys at position 17 is chemically modified by conjugation of the epsilon-amino group of the Lys side chain with (2-[2-(2-amino-ethoxy)-ethoxy]-acetyl)2-(gamma-Glu)-CO-(CH2)16-CO 2H
  SITE 20: note = MISC_FEATURE - Xaa at position 20 is Aib
  SITE 24: note = MISC_FEATURE - Xaa at position 24 is D-Glu
  SITE 25: note = MISC_FEATURE - Xaa at position 25 is alpha-methyl-Tyr
  MOD_RES 39: note = Ser at position 39 is amidated
YXEGTXTSDLSIXLDXKAQXTFIXXLIEGGPSSGAPPPS

SEQ ID NO: 137 - protein, 39 aa, synthetic construct
  REGION 1..39: note = Synthetic Construct
  SITE 2: note = MISC_FEATURE - Xaa at position 2 is Aib
  SITE 6: note = MISC_FEATURE - Xaa at position 6 is alpha-methyl-Phe(2F)
  SITE 13: note = MISC_FEATURE - Xaa at position 13 is alpha-methyl-Leu
  SITE 16: note = MISC_FEATURE - Xaa at position 16 is Orn
  MOD_RES 17: note = Lys at position 17 is chemically modified by conjugation of the epsilon-amino group of the Lys side chain with (2-[2-(2-amino-ethoxy)-ethoxy]-acetyl)2-(gamma-Glu)-CO-(CH2)16-CO 2H
  SITE 20: note = MISC_FEATURE - Xaa at position 20 is Aib
  SITE 24: note = MISC_FEATURE - Xaa at position 24 is D-Glu
  SITE 25: note = MISC_FEATURE - Xaa at position 25 is alpha-methyl-Tyr
  MOD_RES 39: note = Ser at position 39 is amidated
YXEGTXTSDLSIXLDXKAQXAFIXXLIEGGPSSGAPPPS

SEQ ID NO: 138 - protein, 39 aa, synthetic construct
  REGION 1..39: note = Synthetic Construct
  SITE 2: note = MISC_FEATURE - Xaa at position 2 is Aib
  SITE 6: note = MISC_FEATURE - Xaa at position 6 is alpha-methyl-Phe(2F)
  SITE 13: note = MISC_FEATURE - Xaa at position 13 is alpha-methyl-Leu
  SITE 16: note = MISC_FEATURE - Xaa at position 16 is Orn
  MOD_RES 17: note = Lys at position 17 is chemically modified by conjugation of the epsilon-amino group of the Lys side chain with (2-[2-(2-amino-ethoxy)-ethoxy]-acetyl)2-(gamma-Glu)-CO-(CH2)16-CO 2H
  SITE 20: note = MISC_FEATURE - Xaa at position 20 is Aib
  SITE 24: note = MISC_FEATURE - Xaa at position 24 is D-Glu
  SITE 25: note = MISC_FEATURE - Xaa at position 25 is alpha-methyl-Tyr
  MOD_RES 39: note = Ser at position 39 is amidated
YXEGTXTSDASIXLDXKAQXAFIXXLIEGGPSSGAPPPS

SEQ ID NO: 139 - protein, 39 aa, synthetic construct; identical to SEQ ID NO: 11
  REGION 1..39: note = Synthetic Construct
  SITE 2: note = MISC_FEATURE - Xaa at position 2 is Aib
  SITE 6: note = MISC_FEATURE - Xaa at position 6 is alpha-methyl-Phe(2F)
  SITE 13: note = MISC_FEATURE - Xaa at position 13 is Aib
  SITE 16: note = MISC_FEATURE - Xaa at position 16 is Orn
  MOD_RES 17: note = Lys at position 17 is chemically modified by conjugation of the epsilon-amino group of the Lys side chain with (2-[2-(2-amino-ethoxy)-ethoxy]-acetyl)2-(gamma-Glu)-CO-(CH2)16-CO 2H
  SITE 20: note = MISC_FEATURE - Xaa at position 20 is Aib
  SITE 24: note = MISC_FEATURE - Xaa at position 24 is D-Glu
  MOD_RES 39: note = Ser at position 39 is amidated

SEQ ID NO: 140 - protein, 39 aa, synthetic construct
  REGION 1..39: note = Synthetic Construct
  SITE 2: note = MISC_FEATURE - Xaa at position 2 is Aib
  SITE 6: note = MISC_FEATURE - Xaa at position 6 is alpha-methyl-Phe(2F)
  SITE 16: note = MISC_FEATURE - Xaa at position 16 is Orn
  MOD_RES 17: note = Lys at position 17 is chemically modified by conjugation of the epsilon-amino group of the Lys side chain with (2-[2-(2-amino-ethoxy)-ethoxy]-acetyl)2-(gamma-Glu)-CO-(CH2)16-CO 2H
  SITE 20: note = MISC_FEATURE - Xaa at position 20 is Aib
  SITE 24: note = MISC_FEATURE - Xaa at position 24 is D-Glu
  MOD_RES 39: note = Ser at position 39 is amidated
YXEGTXTSDYSILLDXKAQXEFIXYLIEGGPSSGAPPPS

SEQ ID NO: 141 - protein, 39 aa, synthetic construct; identical to SEQ ID NO: 11
  REGION 1..39: note = Synthetic Construct
  SITE 2: note = MISC_FEATURE - Xaa at position 2 is Aib
  SITE 6: note = MISC_FEATURE - Xaa at position 6 is alpha-methyl-Phe(2F)
  SITE 13: note = MISC_FEATURE - Xaa at position 13 is Nle
  SITE 16: note = MISC_FEATURE - Xaa at position 16 is Orn
  MOD_RES 17: note = Lys at position 17 is chemically modified by conjugation of the epsilon-amino group of the Lys side chain with (2-[2-(2-amino-ethoxy)-ethoxy]-acetyl)2-(gamma-Glu)-CO-(CH2)16-CO 2H
  SITE 20: note = MISC_FEATURE - Xaa at position 20 is Aib
  SITE 24: note = MISC_FEATURE - Xaa at position 24 is D-Glu
  MOD_RES 39: note = Ser at position 39 is amidated

SEQ ID NO: 142 - protein, 39 aa, synthetic construct; identical to SEQ ID NO: 11
  REGION 1..39: note = Synthetic Construct
  SITE 2: note = MISC_FEATURE - Xaa at position 2 is Aib
  SITE 6: note = MISC_FEATURE - Xaa at position 6 is alpha-methyl-Phe(2F)
  SITE 13: note = MISC_FEATURE - Xaa at position 13 is Aib
  SITE 16: note = MISC_FEATURE - Xaa at position 16 is Orn
  MOD_RES 17: note = Lys at position 17 is chemically modified by conjugation of the epsilon-amino group of the Lys side chain with (2-[2-(2-amino-ethoxy)-ethoxy]-acetyl)2-(gamma-Glu)-CO-(CH2)18-CO 2H
  SITE 20: note = MISC_FEATURE - Xaa at position 20 is Aib
  SITE 24: note = MISC_FEATURE - Xaa at position 24 is D-Glu
  MOD_RES 39: note = Ser at position 39 is amidated

SEQ ID NO: 143 - protein, 39 aa, synthetic construct
  REGION 1..39: note = Synthetic Construct
  SITE 2: note = MISC_FEATURE - Xaa at position 2 is Aib
  SITE 6: note = MISC_FEATURE - Xaa at position 6 is alpha-methyl-Phe(2F)
  SITE 10: note = MISC_FEATURE - Xaa at position 10 is 4Pal
  SITE 13: note = MISC_FEATURE - Xaa at position 13 is alpha-methyl-Leu
  SITE 16: note = MISC_FEATURE - Xaa at position 16 is Orn
  MOD_RES 17: note = Lys at position 17 is chemically modified by conjugation of the epsilon-amino group of the Lys side chain with (2-[2-(2-amino-ethoxy)-ethoxy]-acetyl)2-(epsilon-Lys)-CO-(CH2)18- CO2H
  SITE 20: note = MISC_FEATURE - Xaa at position 20 is Aib
  SITE 24: note = MISC_FEATURE - Xaa at position 24 is D-Glu
  SITE 25: note = MISC_FEATURE - Xaa at position 25 is alpha-methyl-Tyr
  MOD_RES 39: note = Ser at position 39 is amidated
YXEGTXTSDXSIXLDXKAQXAFIXXLIEGGPSSGAPPPS

SEQ ID NO: 144 - protein, 34 aa, synthetic construct
  REGION 1..34: note = Synthetic Construct
  SITE 2: note = MISC_FEATURE - Xaa at position 2 is Aib
  SITE 6: note = MISC_FEATURE - Xaa at position 6 is alpha-methyl-Phe(2F)
  SITE 10: note = MISC_FEATURE - Xaa at position 10 is 4Pal
  SITE 13: note = MISC_FEATURE - Xaa at position 13 is alpha-methyl-Leu
  SITE 16: note = MISC_FEATURE - Xaa at position 16 is Orn
  MOD_RES 17: note = Lys at position 17 is chemically modified by conjugation of the epsilon-amino group of the Lys side chain with (2-[2-(2-amino-ethoxy)-ethoxy]-acetyl)2-(gamma-Glu)-CO-(CH2)16-CO 2H
  SITE 20: note = MISC_FEATURE - Xaa at position 20 is Aib
  SITE 24: note = MISC_FEATURE - Xaa at position 24 is D-Glu
  SITE 25: note = MISC_FEATURE - Xaa at position 25 is alpha-methyl-Tyr
  MOD_RES 34: note = Gly at position 34 is amidated
YXEGTXTSDXSIXLDXKAQXEFIXXLIEGGPSSG

SEQ ID NO: 145 - protein, 30 aa, synthetic construct
  REGION 1..30: note = Synthetic Construct
  SITE 2: note = MISC_FEATURE - Xaa at position 2 is Aib
  SITE 6: note = MISC_FEATURE - Xaa at position 6 is alpha-methyl-Phe(2F)
  SITE 10: note = MISC_FEATURE - Xaa at position 10 is 4Pal
  SITE 13: note = MISC_FEATURE - Xaa at position 13 is alpha-methyl-Leu
  SITE 16: note = MISC_FEATURE - Xaa at position 13 is Orn
  MOD_RES 17: note = Lys at position 17 is chemically modified by conjugation of the epsilon-amino group of the Lys side chain with (2-[2-(2-amino-ethoxy)-ethoxy]-acetyl)2-(gamma-Glu)-CO-(CH2)16-CO 2H
  SITE 20: note = MISC_FEATURE - Xaa at position 20 is Aib
  SITE 24: note = MISC_FEATURE - Xaa at position 24 is D-Glu
  SITE 25: note = MISC_FEATURE - Xaa at position 25 is alpha-methyl-Tyr
  MOD_RES 30: note = Gly at position 30 is amidated
YXEGTXTSDXSIXLDXKAQXEFIXXLIEGG